European Patent Application EP 4 234 585 A1, published August 30, 2023. Title: FUSION PROTEIN AND APPLICATION THEREOF. Applicant: JIANGSU PROVINCIAL CENTER FOR DISEASE CONTROL AND PREVENTION(PUBLIC HEALTH RESEARCH INSTITUTE OF JIANGSU PROVINCE);Jiangsu Recbio Technology Co., Ltd.;Beijing Abzymo Biosciences Co., Ltd. The sequence listing filed with the application follows.

SEQUENCE LISTING (111 sequences)

SEQ ID NO: 1 - protein, 243 aa, Artificial Sequence
  RBD-P2
RVQPTESIVRFPNITNLCPFGEVFNATRFASVYAWNRKRISNCVADYSVLYNSASFSTFKCYGVSPTKLNDLCFTNVYADSFVIRGDEVRQIAPGQTGKIADYNYKLPDDFTGCVIAWNSNNLDSKVGGNYNYLYRLFRKSNLKPFERDISTEIYQAGSTPCNGVEGFNCYFPLQSYGFQPTNGVGYQPYRVVVLSFELLHAPATVCGPKKSTNLVKNKCVNFGSGSGQYIKANSKFIGITEL

SEQ ID NO: 2 - protein, 243 aa, Artificial Sequence
  P2-RBD
QYIKANSKFIGITELGSGSGRVQPTESIVRFPNITNLCPFGEVFNATRFASVYAWNRKRISNCVADYSVLYNSASFSTFKCYGVSPTKLNDLCFTNVYADSFVIRGDEVRQIAPGQTGKIADYNYKLPDDFTGCVIAWNSNNLDSKVGGNYNYLYRLFRKSNLKPFERDISTEIYQAGSTPCNGVEGFNCYFPLQSYGFQPTNGVGYQPYRVVVLSFELLHAPATVCGPKKSTNLVKNKCVNF

SEQ ID NO: 3 - protein, 255 aa, Artificial Sequence
  RBD-foldon
RVQPTESIVRFPNITNLCPFGEVFNATRFASVYAWNRKRISNCVADYSVLYNSASFSTFKCYGVSPTKLNDLCFTNVYADSFVIRGDEVRQIAPGQTGKIADYNYKLPDDFTGCVIAWNSNNLDSKVGGNYNYLYRLFRKSNLKPFERDISTEIYQAGSTPCNGVEGFNCYFPLQSYGFQPTNGVGYQPYRVVVLSFELLHAPATVCGPKKSTNLVKNKCVNFGSGSGYIPEAPRDGQAYVRKDGEWVLLSTFLG

SEQ ID NO: 4 - protein, 411 aa, Artificial Sequence
  RBD-ferritin LC
RVQPTESIVRFPNITNLCPFGEVFNATRFASVYAWNRKRISNCVADYSVLYNSASFSTFKCYGVSPTKLNDLCFTNVYADSFVIRGDEVRQIAPGQTGKIADYNYKLPDDFTGCVIAWNSNNLDSKVGGNYNYLYRLFRKSNLKPFERDISTEIYQAGSTPCNGVEGFNCYFPLQSYGFQPTNGVGYQPYRVVVLSFELLHAPATVCGPKKSTNLVKNKCVNFGSGSGEYGSHGNVATELQAYAKLHLERSYDYLLSAAYFNNYQTNRAGFSKLFKKLSDEAWSKTIDIIKHVTKRGDKMNFDQHSTMKTERKNYTAENHELEALAKALDTQKELAERAFYIHREATRNSQHLHDPEIAQYLEEEFIEDHAEKIRTLAGHTSDLKKFITANNGHDLSLALYVFDEYLQKTV

SEQ ID NO: 5 - protein, 409 aa, Artificial Sequence
  RBD-ferritin HC
RVQPTESIVRFPNITNLCPFGEVFNATRFASVYAWNRKRISNCVADYSVLYNSASFSTFKCYGVSPTKLNDLCFTNVYADSFVIRGDEVRQIAPGQTGKIADYNYKLPDDFTGCVIAWNSNNLDSKVGGNYNYLYRLFRKSNLKPFERDISTEIYQAGSTPCNGVEGFNCYFPLQSYGFQPTNGVGYQPYRVVVLSFELLHAPATVCGPKKSTNLVKNKCVNFGSGSGRSCRNSMRQQIQMEVGASLQYLAMGAHFSKDVVNRPGFAQLFFDAASEEREHAMKLIEYLLMRGELTNDVSSLLQVRPPTRSSWKGGVEALEHALSMESDVTKSIRNVIKACEDDSEFNDYHLVDYLTGDFLEEQYKGQRDLAGKASTLKKLMDRHEALGEFIFDKKLLGIDVDYKDDDDK

SEQ ID NO: 6 - protein, 454 aa, Artificial Sequence
  RBD-HBsAg
RVQPTESIVRFPNITNLCPFGEVFNATRFASVYAWNRKRISNCVADYSVLYNSASFSTFKCYGVSPTKLNDLCFTNVYADSFVIRGDEVRQIAPGQTGKIADYNYKLPDDFTGCVIAWNSNNLDSKVGGNYNYLYRLFRKSNLKPFERDISTEIYQAGSTPCNGVEGFNCYFPLQSYGFQPTNGVGYQPYRVVVLSFELLHAPATVCGPKKSTNLVKNKCVNFGSGSGMENITSGFLGPLLVLQAGFFLLTRILTIPQSLDSWWTSLNFLGGSPVCLGQNSQSPTSNHSPTSCPPICPGYRWMCLRRFIIFLFILLLCLIFLLVLLDYQGMLPVCPLIPGSTTTSTGPCKTCTTPAQGNSMFPSCCCTKPTDGNCTCIPIPSSWAFAKYLWEWASVRFSWLSLLVPFVQWFVGLSPTVWLSAIWMMWYWGPSLYSIVSPFIPLLPIFFCLWVYI

SEQ ID NO: 7 - protein, 275 aa, Artificial Sequence
  RBD-P2-foldon
RVQPTESIVRFPNITNLCPFGEVFNATRFASVYAWNRKRISNCVADYSVLYNSASFSTFKCYGVSPTKLNDLCFTNVYADSFVIRGDEVRQIAPGQTGKIADYNYKLPDDFTGCVIAWNSNNLDSKVGGNYNYLYRLFRKSNLKPFERDISTEIYQAGSTPCNGVEGFNCYFPLQSYGFQPTNGVGYQPYRVVVLSFELLHAPATVCGPKKSTNLVKNKCVNFGSGSGQYIKANSKFIGITELGSGSGYIPEAPRDGQAYVRKDGEWVLLSTFLG

SEQ ID NO: 8 - protein, 275 aa, Artificial Sequence
  P2-RBD-foldon
QYIKANSKFIGITELGSGSGRVQPTESIVRFPNITNLCPFGEVFNATRFASVYAWNRKRISNCVADYSVLYNSASFSTFKCYGVSPTKLNDLCFTNVYADSFVIRGDEVRQIAPGQTGKIADYNYKLPDDFTGCVIAWNSNNLDSKVGGNYNYLYRLFRKSNLKPFERDISTEIYQAGSTPCNGVEGFNCYFPLQSYGFQPTNGVGYQPYRVVVLSFELLHAPATVCGPKKSTNLVKNKCVNFGSGSGYIPEAPRDGQAYVRKDGEWVLLSTFLG

SEQ ID NO: 9 - protein, 275 aa, Artificial Sequence
  RBD-foldon-P2
RVQPTESIVRFPNITNLCPFGEVFNATRFASVYAWNRKRISNCVADYSVLYNSASFSTFKCYGVSPTKLNDLCFTNVYADSFVIRGDEVRQIAPGQTGKIADYNYKLPDDFTGCVIAWNSNNLDSKVGGNYNYLYRLFRKSNLKPFERDISTEIYQAGSTPCNGVEGFNCYFPLQSYGFQPTNGVGYQPYRVVVLSFELLHAPATVCGPKKSTNLVKNKCVNFGSGSGYIPEAPRDGQAYVRKDGEWVLLSTFLGGSGSGQYIKANSKFIGITEL

SEQ ID NO: 10 - protein, 431 aa, Artificial Sequence
  RBD-P2-ferritin LC
RVQPTESIVRFPNITNLCPFGEVFNATRFASVYAWNRKRISNCVADYSVLYNSASFSTFKCYGVSPTKLNDLCFTNVYADSFVIRGDEVRQIAPGQTGKIADYNYKLPDDFTGCVIAWNSNNLDSKVGGNYNYLYRLFRKSNLKPFERDISTEIYQAGSTPCNGVEGFNCYFPLQSYGFQPTNGVGYQPYRVVVLSFELLHAPATVCGPKKSTNLVKNKCVNFGSGSGQYIKANSKFIGITELGSGSGEYGSHGNVATELQAYAKLHLERSYDYLLSAAYFNNYQTNRAGFSKLFKKLSDEAWSKTIDIIKHVTKRGDKMNFDQHSTMKTERKNYTAENHELEALAKALDTQKELAERAFYIHREATRNSQHLHDPEIAQYLEEEFIEDHAEKIRTLAGHTSDLKKFITANNGHDLSLALYVFDEYLQKTV

SEQ ID NO: 11 - protein, 429 aa, Artificial Sequence
  RBD-P2-ferritin HC
RVQPTESIVRFPNITNLCPFGEVFNATRFASVYAWNRKRISNCVADYSVLYNSASFSTFKCYGVSPTKLNDLCFTNVYADSFVIRGDEVRQIAPGQTGKIADYNYKLPDDFTGCVIAWNSNNLDSKVGGNYNYLYRLFRKSNLKPFERDISTEIYQAGSTPCNGVEGFNCYFPLQSYGFQPTNGVGYQPYRVVVLSFELLHAPATVCGPKKSTNLVKNKCVNFGSGSGQYIKANSKFIGITELGSGSGRSCRNSMRQQIQMEVGASLQYLAMGAHFSKDVVNRPGFAQLFFDAASEEREHAMKLIEYLLMRGELTNDVSSLLQVRPPTRSSWKGGVEALEHALSMESDVTKSIRNVIKACEDDSEFNDYHLVDYLTGDFLEEQYKGQRDLAGKASTLKKLMDRHEALGEFIFDKKLLGIDVDYKDDDDK

SEQ ID NO: 12 - protein, 431 aa, Artificial Sequence
  P2-RBD-ferritin LC
QYIKANSKFIGITELGSGSGRVQPTESIVRFPNITNLCPFGEVFNATRFASVYAWNRKRISNCVADYSVLYNSASFSTFKCYGVSPTKLNDLCFTNVYADSFVIRGDEVRQIAPGQTGKIADYNYKLPDDFTGCVIAWNSNNLDSKVGGNYNYLYRLFRKSNLKPFERDISTEIYQAGSTPCNGVEGFNCYFPLQSYGFQPTNGVGYQPYRVVVLSFELLHAPATVCGPKKSTNLVKNKCVNFGSGSGEYGSHGNVATELQAYAKLHLERSYDYLLSAAYFNNYQTNRAGFSKLFKKLSDEAWSKTIDIIKHVTKRGDKMNFDQHSTMKTERKNYTAENHELEALAKALDTQKELAERAFYIHREATRNSQHLHDPEIAQYLEEEFIEDHAEKIRTLAGHTSDLKKFITANNGHDLSLALYVFDEYLQKTV

SEQ ID NO: 13 - protein, 429 aa, Artificial Sequence
  P2-RBD-ferritin HC
QYIKANSKFIGITELGSGSGRVQPTESIVRFPNITNLCPFGEVFNATRFASVYAWNRKRISNCVADYSVLYNSASFSTFKCYGVSPTKLNDLCFTNVYADSFVIRGDEVRQIAPGQTGKIADYNYKLPDDFTGCVIAWNSNNLDSKVGGNYNYLYRLFRKSNLKPFERDISTEIYQAGSTPCNGVEGFNCYFPLQSYGFQPTNGVGYQPYRVVVLSFELLHAPATVCGPKKSTNLVKNKCVNFGSGSGRSCRNSMRQQIQMEVGASLQYLAMGAHFSKDVVNRPGFAQLFFDAASEEREHAMKLIEYLLMRGELTNDVSSLLQVRPPTRSSWKGGVEALEHALSMESDVTKSIRNVIKACEDDSEFNDYHLVDYLTGDFLEEQYKGQRDLAGKASTLKKLMDRHEALGEFIFDKKLLGIDVDYKDDDDK

SEQ ID NO: 14 - protein, 411 aa, Artificial Sequence
  P2-RBD-ferritin
QYIKANSKFIGITELGSGSGRVQPTESIVRFPNITNLCPFGEVFNATRFASVYAWNRKRISNCVADYSVLYNSASFSTFKCYGVSPTKLNDLCFTNVYADSFVIRGDEVRQIAPGQTGKIADYNYKLPDDFTGCVIAWNSNNLDSKVGGNYNYLYRLFRKSNLKPFERDISTEIYQAGSTPCNGVEGFNCYFPLQSYGFQPTNGVGYQPYRVVVLSFELLHAPATVCGPKKSTNLVKNKCVNFGSGSGDIIKLLNEQVNKEMNSSNLYMSMSSWCYTHSLDGAGLFLFDHAAEEYEHAKKLIIFLNENNVPVQLTSISAPEHKFEGLTQIFQKAYEHEQHISESINNIVDHAIKSKDHATFNFLQWYVAEQHEEEVLFKDILDKIELIGNENHGLYLADQYVKGIAKSRKS

SEQ ID NO: 15 - protein, 474 aa, Artificial Sequence
  RBD-P2-HBsAg
RVQPTESIVRFPNITNLCPFGEVFNATRFASVYAWNRKRISNCVADYSVLYNSASFSTFKCYGVSPTKLNDLCFTNVYADSFVIRGDEVRQIAPGQTGKIADYNYKLPDDFTGCVIAWNSNNLDSKVGGNYNYLYRLFRKSNLKPFERDISTEIYQAGSTPCNGVEGFNCYFPLQSYGFQPTNGVGYQPYRVVVLSFELLHAPATVCGPKKSTNLVKNKCVNFGSGSGQYIKANSKFIGITELGSGSGMENITSGFLGPLLVLQAGFFLLTRILTIPQSLDSWWTSLNFLGGSPVCLGQNSQSPTSNHSPTSCPPICPGYRWMCLRRFIIFLFILLLCLIFLLVLLDYQGMLPVCPLIPGSTTTSTGPCKTCTTPAQGNSMFPSCCCTKPTDGNCTCIPIPSSWAFAKYLWEWASVRFSWLSLLVPFVQWFVGLSPTVWLSAIWMMWYWGPSLYSIVSPFIPLLPIFFCLWVYI

SEQ ID NO: 16 - protein, 474 aa, Artificial Sequence
  P2-RBD-HBsAg
QYIKANSKFIGITELGSGSGRVQPTESIVRFPNITNLCPFGEVFNATRFASVYAWNRKRISNCVADYSVLYNSASFSTFKCYGVSPTKLNDLCFTNVYADSFVIRGDEVRQIAPGQTGKIADYNYKLPDDFTGCVIAWNSNNLDSKVGGNYNYLYRLFRKSNLKPFERDISTEIYQAGSTPCNGVEGFNCYFPLQSYGFQPTNGVGYQPYRVVVLSFELLHAPATVCGPKKSTNLVKNKCVNFGSGSGMENITSGFLGPLLVLQAGFFLLTRILTIPQSLDSWWTSLNFLGGSPVCLGQNSQSPTSNHSPTSCPPICPGYRWMCLRRFIIFLFILLLCLIFLLVLLDYQGMLPVCPLIPGSTTTSTGPCKTCTTPAQGNSMFPSCCCTKPTDGNCTCIPIPSSWAFAKYLWEWASVRFSWLSLLVPFVQWFVGLSPTVWLSAIWMMWYWGPSLYSIVSPFIPLLPIFFCLWVYI

SEQ ID NO: 17 - protein, 474 aa, Artificial Sequence
  RBD-HBsAg-P2
RVQPTESIVRFPNITNLCPFGEVFNATRFASVYAWNRKRISNCVADYSVLYNSASFSTFKCYGVSPTKLNDLCFTNVYADSFVIRGDEVRQIAPGQTGKIADYNYKLPDDFTGCVIAWNSNNLDSKVGGNYNYLYRLFRKSNLKPFERDISTEIYQAGSTPCNGVEGFNCYFPLQSYGFQPTNGVGYQPYRVVVLSFELLHAPATVCGPKKSTNLVKNKCVNFGSGSGMENITSGFLGPLLVLQAGFFLLTRILTIPQSLDSWWTSLNFLGGSPVCLGQNSQSPTSNHSPTSCPPICPGYRWMCLRRFIIFLFILLLCLIFLLVLLDYQGMLPVCPLIPGSTTTSTGPCKTCTTPAQGNSMFPSCCCTKPTDGNCTCIPIPSSWAFAKYLWEWASVRFSWLSLLVPFVQWFVGLSPTVWLSAIWMMWYWGPSLYSIVSPFIPLLPIFFCLWVYIGSGSGQYIKANSKFIGITEL

SEQ ID NO: 18 - protein, 223 aa, Artificial Sequence
  RBD 319-541
RVQPTESIVRFPNITNLCPFGEVFNATRFASVYAWNRKRISNCVADYSVLYNSASFSTFKCYGVSPTKLNDLCFTNVYADSFVIRGDEVRQIAPGQTGKIADYNYKLPDDFTGCVIAWNSNNLDSKVGGNYNYLYRLFRKSNLKPFERDISTEIYQAGSTPCNGVEGFNCYFPLQSYGFQPTNGVGYQPYRVVVLSFELLHAPATVCGPKKSTNLVKNKCVNF

SEQ ID NO: 19 - protein, 194 aa, Artificial Sequence
  RBD 331-524
NITNLCPFGEVFNATRFASVYAWNRKRISNCVADYSVLYNSASFSTFKCYGVSPTKLNDLCFTNVYADSFVIRGDEVRQIAPGQTGKIADYNYKLPDDFTGCVIAWNSNNLDSKVGGNYNYLYRLFRKSNLKPFERDISTEIYQAGSTPCNGVEGFNCYFPLQSYGFQPTNGVGYQPYRVVVLSFELLHAPATV

SEQ ID NO: 20 - protein, 311 aa, Artificial Sequence
  NTD-P2
QCVNLTTRTQLPPAYTNSFTRGVYYPDKVFRSSVLHSTQDLFLPFFSNVTWFHAIHVSGTNGTKRFDNPVLPFNDGVYFASTEKSNIIRGWIFGTTLDSKTQSLLIVNNATNVVIKVCEFQFCNDPFLGVYYHKNNKSWMESEFRVYSSANNCTFEYVSQPFLMDLEGKQGNFKNLREFVFKNIDGYFKIYSKHTPINLVRDLPQGFSALEPLVDLPIGINITRFQTLLALHRSYLTPGDSSSGWTAGAAAYYVGYLQPRTFLLKYNENGTITDAVDCALDPLSETKCTLKGSGSGQYIKANSKFIGITEL

SEQ ID NO: 21 - protein, 311 aa, Artificial Sequence
  P2-NTD
QYIKANSKFIGITELGSGSGQCVNLTTRTQLPPAYTNSFTRGVYYPDKVFRSSVLHSTQDLFLPFFSNVTWFHAIHVSGTNGTKRFDNPVLPFNDGVYFASTEKSNIIRGWIFGTTLDSKTQSLLIVNNATNVVIKVCEFQFCNDPFLGVYYHKNNKSWMESEFRVYSSANNCTFEYVSQPFLMDLEGKQGNFKNLREFVFKNIDGYFKIYSKHTPINLVRDLPQGFSALEPLVDLPIGINITRFQTLLALHRSYLTPGDSSSGWTAGAAAYYVGYLQPRTFLLKYNENGTITDAVDCALDPLSETKCTLK

SEQ ID NO: 22 - protein, 323 aa, Artificial Sequence
  NTD-foldon
QCVNLTTRTQLPPAYTNSFTRGVYYPDKVFRSSVLHSTQDLFLPFFSNVTWFHAIHVSGTNGTKRFDNPVLPFNDGVYFASTEKSNIIRGWIFGTTLDSKTQSLLIVNNATNVVIKVCEFQFCNDPFLGVYYHKNNKSWMESEFRVYSSANNCTFEYVSQPFLMDLEGKQGNFKNLREFVFKNIDGYFKIYSKHTPINLVRDLPQGFSALEPLVDLPIGINITRFQTLLALHRSYLTPGDSSSGWTAGAAAYYVGYLQPRTFLLKYNENGTITDAVDCALDPLSETKCTLKGSGSGYIPEAPRDGQAYVRKDGEWVLLSTFLG

SEQ ID NO: 23 - protein, 478 aa, Artificial Sequence
  NTD-ferritin LC
QCVNLTTRTQLPPAYTNSFTRGVYYPDKVFRSSVLHSTQDLFLPFFSNVTWFHAIHVSGTNGTKRFDNPVLPFNDGVYFASTEKSNIIRGWIFGTTLDSKTQSLLIVNNATNVVIKVCEFQFCNDPFLGVYYHKNNKSWMESEFRVYSSANNCTFEYVSQPFLMDLEGKQGNFKNLREFVFKNIDGYFKIYSKHTPINLVRDLPQGFSALEPLVDLPIGINITRFQTLLALHRSYLTPGDSSSGWTAGAAAYYVGYLQPRTFLLKYNENGTITDAVDCALDPLSETKCTLGSGSGEYGSHGNVATELQAYAKLHLERSYDYLLSAAYFNNYQTNRAGFSKLFKKLSDEAWSKTIDIIKHVTKRGDKMNFDQHSTMKTERKNYTAENHELEALAKALDTQKELAERAFYIHREATRNSQHLHDPEIAQYLEEEFIEDHAEKIRTLAGHTSDLKKFITANNGHDLSLALYVFDEYLQKTV

SEQ ID NO: 24 - protein, 476 aa, Artificial Sequence
  NTD-ferritin HC
QCVNLTTRTQLPPAYTNSFTRGVYYPDKVFRSSVLHSTQDLFLPFFSNVTWFHAIHVSGTNGTKRFDNPVLPFNDGVYFASTEKSNIIRGWIFGTTLDSKTQSLLIVNNATNVVIKVCEFQFCNDPFLGVYYHKNNKSWMESEFRVYSSANNCTFEYVSQPFLMDLEGKQGNFKNLREFVFKNIDGYFKIYSKHTPINLVRDLPQGFSALEPLVDLPIGINITRFQTLLALHRSYLTPGDSSSGWTAGAAAYYVGYLQPRTFLLKYNENGTITDAVDCALDPLSETKCTLGSGSGRSCRNSMRQQIQMEVGASLQYLAMGAHFSKDVVNRPGFAQLFFDAASEEREHAMKLIEYLLMRGELTNDVSSLLQVRPPTRSSWKGGVEALEHALSMESDVTKSIRNVIKACEDDSEFNDYHLVDYLTGDFLEEQYKGQRDLAGKASTLKKLMDRHEALGEFIFDKKLLGIDVDYKDDDDK

SEQ ID NO: 25 - protein, 521 aa, Artificial Sequence
  NTD-HBsAg
QCVNLTTRTQLPPAYTNSFTRGVYYPDKVFRSSVLHSTQDLFLPFFSNVTWFHAIHVSGTNGTKRFDNPVLPFNDGVYFASTEKSNIIRGWIFGTTLDSKTQSLLIVNNATNVVIKVCEFQFCNDPFLGVYYHKNNKSWMESEFRVYSSANNCTFEYVSQPFLMDLEGKQGNFKNLREFVFKNIDGYFKIYSKHTPINLVRDLPQGFSALEPLVDLPIGINITRFQTLLALHRSYLTPGDSSSGWTAGAAAYYVGYLQPRTFLLKYNENGTITDAVDCALDPLSETKCTLGSGSGMENITSGFLGPLLVLQAGFFLLTRILTIPQSLDSWWTSLNFLGGSPVCLGQNSQSPTSNHSPTSCPPICPGYRWMCLRRFIIFLFILLLCLIFLLVLLDYQGMLPVCPLIPGSTTTSTGPCKTCTTPAQGNSMFPSCCCTKPTDGNCTCIPIPSSWAFAKYLWEWASVRFSWLSLLVPFVQWFVGLSPTVWLSAIWMMWYWGPSLYSIVSPFIPLLPIFFCLWVYI

SEQ ID NO: 26 - protein, 342 aa, Artificial Sequence
  NTD-P2-foldon
QCVNLTTRTQLPPAYTNSFTRGVYYPDKVFRSSVLHSTQDLFLPFFSNVTWFHAIHVSGTNGTKRFDNPVLPFNDGVYFASTEKSNIIRGWIFGTTLDSKTQSLLIVNNATNVVIKVCEFQFCNDPFLGVYYHKNNKSWMESEFRVYSSANNCTFEYVSQPFLMDLEGKQGNFKNLREFVFKNIDGYFKIYSKHTPINLVRDLPQGFSALEPLVDLPIGINITRFQTLLALHRSYLTPGDSSSGWTAGAAAYYVGYLQPRTFLLKYNENGTITDAVDCALDPLSETKCTLGSGSGQYIKANSKFIGITELGSGSGYIPEAPRDGQAYVRKDGEWVLLSTFLG

SEQ ID NO: 27 - protein, 342 aa, Artificial Sequence
  P2-NTD-foldon
QYIKANSKFIGITELGSGSGQCVNLTTRTQLPPAYTNSFTRGVYYPDKVFRSSVLHSTQDLFLPFFSNVTWFHAIHVSGTNGTKRFDNPVLPFNDGVYFASTEKSNIIRGWIFGTTLDSKTQSLLIVNNATNVVIKVCEFQFCNDPFLGVYYHKNNKSWMESEFRVYSSANNCTFEYVSQPFLMDLEGKQGNFKNLREFVFKNIDGYFKIYSKHTPINLVRDLPQGFSALEPLVDLPIGINITRFQTLLALHRSYLTPGDSSSGWTAGAAAYYVGYLQPRTFLLKYNENGTITDAVDCALDPLSETKCTLGSGSGYIPEAPRDGQAYVRKDGEWVLLSTFLG

SEQ ID NO: 28 - protein, 342 aa, Artificial Sequence
  NTD-foldon-P2
QCVNLTTRTQLPPAYTNSFTRGVYYPDKVFRSSVLHSTQDLFLPFFSNVTWFHAIHVSGTNGTKRFDNPVLPFNDGVYFASTEKSNIIRGWIFGTTLDSKTQSLLIVNNATNVVIKVCEFQFCNDPFLGVYYHKNNKSWMESEFRVYSSANNCTFEYVSQPFLMDLEGKQGNFKNLREFVFKNIDGYFKIYSKHTPINLVRDLPQGFSALEPLVDLPIGINITRFQTLLALHRSYLTPGDSSSGWTAGAAAYYVGYLQPRTFLLKYNENGTITDAVDCALDPLSETKCTLGSGSGYIPEAPRDGQAYVRKDGEWVLLSTFLGGSGSGQYIKANSKFIGITEL

SEQ ID NO: 29 - protein, 498 aa, Artificial Sequence
  NTD-P2-ferritin LC
QCVNLTTRTQLPPAYTNSFTRGVYYPDKVFRSSVLHSTQDLFLPFFSNVTWFHAIHVSGTNGTKRFDNPVLPFNDGVYFASTEKSNIIRGWIFGTTLDSKTQSLLIVNNATNVVIKVCEFQFCNDPFLGVYYHKNNKSWMESEFRVYSSANNCTFEYVSQPFLMDLEGKQGNFKNLREFVFKNIDGYFKIYSKHTPINLVRDLPQGFSALEPLVDLPIGINITRFQTLLALHRSYLTPGDSSSGWTAGAAAYYVGYLQPRTFLLKYNENGTITDAVDCALDPLSETKCTLGSGSGQYIKANSKFIGITELGSGSGEYGSHGNVATELQAYAKLHLERSYDYLLSAAYFNNYQTNRAGFSKLFKKLSDEAWSKTIDIIKHVTKRGDKMNFDQHSTMKTERKNYTAENHELEALAKALDTQKELAERAFYIHREATRNSQHLHDPEIAQYLEEEFIEDHAEKIRTLAGHTSDLKKFITANNGHDLSLALYVFDEYLQKTV

SEQ ID NO: 30 - protein, 488 aa, Artificial Sequence
  NTD-P2-ferritin HC
QCVNLTTRTQLPPAYTNSFTRGVYYPDKVFRSSVLHSTQDLFLPFFSNVTWFHAIHVSGTNGTKRFDNPVLPFNDGVYFASTEKSNIIRGWIFGTTLDSKTQSLLIVNNATNVVIKVCEFQFCNDPFLGVYYHKNNKSWMESEFRVYSSANNCTFEYVSQPFLMDLEGKQGNFKNLREFVFKNIDGYFKIYSKHTPINLVRDLPQGFSALEPLVDLPIGINITRFQTLLALHRSYLTPGDSSSGWTAGAAAYYVGYLQPRTFLLKYNENGTITDAVDCALDPLSETKCTLGSGSGQYIKANSKFIGITELGSGSGRSCRNSMRQQIQMEVGASLQYLAMGAHFSKDVVNRPGFAQLFFDAASEEREHAMKLIEYLLMRGELTNDVSSLLQVRPPTRSSWKGGVEALEHALSMESDVTKSIRNVIKACEDDSEFNDYHLVDYLTGDFLEEQYKGQRDLAGKASTLKKLMDRHEALGEFIFDKKLLGIDV

SEQ ID NO: 31 - protein, 498 aa, Artificial Sequence
  P2-NTD-ferritin LC
QYIKANSKFIGITELGSGSGQCVNLTTRTQLPPAYTNSFTRGVYYPDKVFRSSVLHSTQDLFLPFFSNVTWFHAIHVSGTNGTKRFDNPVLPFNDGVYFASTEKSNIIRGWIFGTTLDSKTQSLLIVNNATNVVIKVCEFQFCNDPFLGVYYHKNNKSWMESEFRVYSSANNCTFEYVSQPFLMDLEGKQGNFKNLREFVFKNIDGYFKIYSKHTPINLVRDLPQGFSALEPLVDLPIGINITRFQTLLALHRSYLTPGDSSSGWTAGAAAYYVGYLQPRTFLLKYNENGTITDAVDCALDPLSETKCTLGSGSGEYGSHGNVATELQAYAKLHLERSYDYLLSAAYFNNYQTNRAGFSKLFKKLSDEAWSKTIDIIKHVTKRGDKMNFDQHSTMKTERKNYTAENHELEALAKALDTQKELAERAFYIHREATRNSQHLHDPEIAQYLEEEFIEDHAEKIRTLAGHTSDLKKFITANNGHDLSLALYVFDEYLQKTV

SEQ ID NO: 32 - protein, 488 aa, Artificial Sequence
  P2-NTD-ferritin HC
QYIKANSKFIGITELGSGSGQCVNLTTRTQLPPAYTNSFTRGVYYPDKVFRSSVLHSTQDLFLPFFSNVTWFHAIHVSGTNGTKRFDNPVLPFNDGVYFASTEKSNIIRGWIFGTTLDSKTQSLLIVNNATNVVIKVCEFQFCNDPFLGVYYHKNNKSWMESEFRVYSSANNCTFEYVSQPFLMDLEGKQGNFKNLREFVFKNIDGYFKIYSKHTPINLVRDLPQGFSALEPLVDLPIGINITRFQTLLALHRSYLTPGDSSSGWTAGAAAYYVGYLQPRTFLLKYNENGTITDAVDCALDPLSETKCTLGSGSGRSCRNSMRQQIQMEVGASLQYLAMGAHFSKDVVNRPGFAQLFFDAASEEREHAMKLIEYLLMRGELTNDVSSLLQVRPPTRSSWKGGVEALEHALSMESDVTKSIRNVIKACEDDSEFNDYHLVDYLTGDFLEEQYKGQRDLAGKASTLKKLMDRHEALGEFIFDKKLLGIDV

SEQ ID NO: 33 - protein, 478 aa, Artificial Sequence
  P2-NTD-ferritin
QYIKANSKFIGITELGSGSGQCVNLTTRTQLPPAYTNSFTRGVYYPDKVFRSSVLHSTQDLFLPFFSNVTWFHAIHVSGTNGTKRFDNPVLPFNDGVYFASTEKSNIIRGWIFGTTLDSKTQSLLIVNNATNVVIKVCEFQFCNDPFLGVYYHKNNKSWMESEFRVYSSANNCTFEYVSQPFLMDLEGKQGNFKNLREFVFKNIDGYFKIYSKHTPINLVRDLPQGFSALEPLVDLPIGINITRFQTLLALHRSYLTPGDSSSGWTAGAAAYYVGYLQPRTFLLKYNENGTITDAVDCALDPLSETKCTLGSGSGDIIKLLNEQVNKEMNSSNLYMSMSSWCYTHSLDGAGLFLFDHAAEEYEHAKKLIIFLNENNVPVQLTSISAPEHKFEGLTQIFQKAYEHEQHISESINNIVDHAIKSKDHATFNFLQWYVAEQHEEEVLFKDILDKIELIGNENHGLYLADQYVKGIAKSRKS

SEQ ID NO: 34 - protein, 541 aa, Artificial Sequence
  NTD-P2-HBsAg
QCVNLTTRTQLPPAYTNSFTRGVYYPDKVFRSSVLHSTQDLFLPFFSNVTWFHAIHVSGTNGTKRFDNPVLPFNDGVYFASTEKSNIIRGWIFGTTLDSKTQSLLIVNNATNVVIKVCEFQFCNDPFLGVYYHKNNKSWMESEFRVYSSANNCTFEYVSQPFLMDLEGKQGNFKNLREFVFKNIDGYFKIYSKHTPINLVRDLPQGFSALEPLVDLPIGINITRFQTLLALHRSYLTPGDSSSGWTAGAAAYYVGYLQPRTFLLKYNENGTITDAVDCALDPLSETKCTLGSGSGQYIKANSKFIGITELGSGSGMENITSGFLGPLLVLQAGFFLLTRILTIPQSLDSWWTSLNFLGGSPVCLGQNSQSPTSNHSPTSCPPICPGYRWMCLRRFIIFLFILLLCLIFLLVLLDYQGMLPVCPLIPGSTTTSTGPCKTCTTPAQGNSMFPSCCCTKPTDGNCTCIPIPSSWAFAKYLWEWASVRFSWLSLLVPFVQWFVGLSPTVWLSAIWMMWYWGPSLYSIVSPFIPLLPIFFCLWVYI

SEQ ID NO: 35 - protein, 541 aa, Artificial Sequence
  P2-NTD-HBsAg
QYIKANSKFIGITELGSGSGQCVNLTTRTQLPPAYTNSFTRGVYYPDKVFRSSVLHSTQDLFLPFFSNVTWFHAIHVSGTNGTKRFDNPVLPFNDGVYFASTEKSNIIRGWIFGTTLDSKTQSLLIVNNATNVVIKVCEFQFCNDPFLGVYYHKNNKSWMESEFRVYSSANNCTFEYVSQPFLMDLEGKQGNFKNLREFVFKNIDGYFKIYSKHTPINLVRDLPQGFSALEPLVDLPIGINITRFQTLLALHRSYLTPGDSSSGWTAGAAAYYVGYLQPRTFLLKYNENGTITDAVDCALDPLSETKCTLGSGSGMENITSGFLGPLLVLQAGFFLLTRILTIPQSLDSWWTSLNFLGGSPVCLGQNSQSPTSNHSPTSCPPICPGYRWMCLRRFIIFLFILLLCLIFLLVLLDYQGMLPVCPLIPGSTTTSTGPCKTCTTPAQGNSMFPSCCCTKPTDGNCTCIPIPSSWAFAKYLWEWASVRFSWLSLLVPFVQWFVGLSPTVWLSAIWMMWYWGPSLYSIVSPFIPLLPIFFCLWVYI

SEQ ID NO: 36 - protein, 541 aa, Artificial Sequence
  NTD-HBsAg-P2
QCVNLTTRTQLPPAYTNSFTRGVYYPDKVFRSSVLHSTQDLFLPFFSNVTWFHAIHVSGTNGTKRFDNPVLPFNDGVYFASTEKSNIIRGWIFGTTLDSKTQSLLIVNNATNVVIKVCEFQFCNDPFLGVYYHKNNKSWMESEFRVYSSANNCTFEYVSQPFLMDLEGKQGNFKNLREFVFKNIDGYFKIYSKHTPINLVRDLPQGFSALEPLVDLPIGINITRFQTLLALHRSYLTPGDSSSGWTAGAAAYYVGYLQPRTFLLKYNENGTITDAVDCALDPLSETKCTLGSGSGMENITSGFLGPLLVLQAGFFLLTRILTIPQSLDSWWTSLNFLGGSPVCLGQNSQSPTSNHSPTSCPPICPGYRWMCLRRFIIFLFILLLCLIFLLVLLDYQGMLPVCPLIPGSTTTSTGPCKTCTTPAQGNSMFPSCCCTKPTDGNCTCIPIPSSWAFAKYLWEWASVRFSWLSLLVPFVQWFVGLSPTVWLSAIWMMWYWGPSLYSIVSPFIPLLPIFFCLWVYIGSGSGQYIKANSKFIGITEL

SEQ ID NO: 37 - protein, 291 aa, Artificial Sequence
  NTD 14-304
QCVNLTTRTQLPPAYTNSFTRGVYYPDKVFRSSVLHSTQDLFLPFFSNVTWFHAIHVSGTNGTKRFDNPVLPFNDGVYFASTEKSNIIRGWIFGTTLDSKTQSLLIVNNATNVVIKVCEFQFCNDPFLGVYYHKNNKSWMESEFRVYSSANNCTFEYVSQPFLMDLEGKQGNFKNLREFVFKNIDGYFKIYSKHTPINLVRDLPQGFSALEPLVDLPIGINITRFQTLLALHRSYLTPGDSSSGWTAGAAAYYVGYLQPRTFLLKYNENGTITDAVDCALDPLSETKCTLK

SEQ ID NO: 38 - protein, 336 aa, Artificial Sequence
  NTD 18-353
LTTRTQLPPAYTNSFTRGVYYPDKVFRSSVLHSTQDLFLPFFSNVTWFHAIHVSGTNGTKRFDNPVLPFNDGVYFASTEKSNIIRGWIFGTTLDSKTQSLLIVNNATNVVIKVCEFQFCNDPFLGVYYHKNNKSWMESEFRVYSSANNCTFEYVSQPFLMDLEGKQGNFKNLREFVFKNIDGYFKIYSKHTPINLVRDLPQGFSALEPLVDLPIGINITRFQTLLALHRSYLTPGDSSSGWTAGAAAYYVGYLQPRTFLLKYNENGTITDAVDCALDPLSETKCTLKSFTVEKGIYQTSNFRVQPTESIVRFPNITNLCPFGEVFNATRFASVYAW

SEQ ID NO: 39 - protein, 536 aa, Artificial Sequence
  NTD-RBD-6His
QCVNLTTRTQLPPAYTNSFTRGVYYPDKVFRSSVLHSTQDLFLPFFSNVTWFHAIHVSGTNGTKRFDNPVLPFNDGVYFASTEKSNIIRGWIFGTTLDSKTQSLLIVNNATNVVIKVCEFQFCNDPFLGVYYHKNNKSWMESEFRVYSSANNCTFEYVSQPFLMDLEGKQGNFKNLREFVFKNIDGYFKIYSKHTPINLVRDLPQGFSALEPLVDLPIGINITRFQTLLALHRSYLTPGDSSSGWTAGAAAYYVGYLQPRTFLLKYNENGTITDAVDCALDPLSETKCTLKSFTVEKGIYQTSNFRVQPTESIVRFPNITNLCPFGEVFNATRFASVYAWNRKRISNCVADYSVLYNSASFSTFKCYGVSPTKLNDLCFTNVYADSFVIRGDEVRQIAPGQTGKIADYNYKLPDDFTGCVIAWNSNNLDSKVGGNYNYLYRLFRKSNLKPFERDISTEIYQAGSTPCNGVEGFNCYFPLQSYGFQPTNGVGYQPYRVVVLSFELLHAPATVCGPKKSTNLVKNKCVNFGSHHHHHH

SEQ ID NO: 40 - protein, 556 aa, Artificial Sequence
  NTD-RBD-P2-6His
QCVNLTTRTQLPPAYTNSFTRGVYYPDKVFRSSVLHSTQDLFLPFFSNVTWFHAIHVSGTNGTKRFDNPVLPFNDGVYFASTEKSNIIRGWIFGTTLDSKTQSLLIVNNATNVVIKVCEFQFCNDPFLGVYYHKNNKSWMESEFRVYSSANNCTFEYVSQPFLMDLEGKQGNFKNLREFVFKNIDGYFKIYSKHTPINLVRDLPQGFSALEPLVDLPIGINITRFQTLLALHRSYLTPGDSSSGWTAGAAAYYVGYLQPRTFLLKYNENGTITDAVDCALDPLSETKCTLKSFTVEKGIYQTSNFRVQPTESIVRFPNITNLCPFGEVFNATRFASVYAWNRKRISNCVADYSVLYNSASFSTFKCYGVSPTKLNDLCFTNVYADSFVIRGDEVRQIAPGQTGKIADYNYKLPDDFTGCVIAWNSNNLDSKVGGNYNYLYRLFRKSNLKPFERDISTEIYQAGSTPCNGVEGFNCYFPLQSYGFQPTNGVGYQPYRVVVLSFELLHAPATVCGPKKSTNLVKNKCVNFGSGSGQYIKANSKFIGITELGSHHHHHH

SEQ ID NO: 41 - protein, 588 aa, Artificial Sequence
  NTD-RBD-foldon-6His
MKHLWFFLLLVAAPRWVLSSQCVNLTTRTQLPPAYTNSFTRGVYYPDKVFRSSVLHSTQDLFLPFFSNVTWFHAIHVSGTNGTKRFDNPVLPFNDGVYFASTEKSNIIRGWIFGTTLDSKTQSLLIVNNATNVVIKVCEFQFCNDPFLGVYYHKNNKSWMESEFRVYSSANNCTFEYVSQPFLMDLEGKQGNFKNLREFVFKNIDGYFKIYSKHTPINLVRDLPQGFSALEPLVDLPIGINITRFQTLLALHRSYLTPGDSSSGWTAGAAAYYVGYLQPRTFLLKYNENGTITDAVDCALDPLSETKCTLKSFTVEKGIYQTSNFRVQPTESIVRFPNITNLCPFGEVFNATRFASVYAWNRKRISNCVADYSVLYNSASFSTFKCYGVSPTKLNDLCFTNVYADSFVIRGDEVRQIAPGQTGKIADYNYKLPDDFTGCVIAWNSNNLDSKVGGNYNYLYRLFRKSNLKPFERDISTEIYQAGSTPCNGVEGFNCYFPLQSYGFQPTNGVGYQPYRVVVLSFELLHAPATVCGPKKSTNLVKNKCVNFGSGSGYIPEAPRDGQAYVRKDGEWVLLSTFLGGSHHHHHH

SEQ ID NO: 42 - protein, 608 aa, Artificial Sequence
  NTD-RBD-P2-foldon-6His
MKHLWFFLLLVAAPRWVLSSQCVNLTTRTQLPPAYTNSFTRGVYYPDKVFRSSVLHSTQDLFLPFFSNVTWFHAIHVSGTNGTKRFDNPVLPFNDGVYFASTEKSNIIRGWIFGTTLDSKTQSLLIVNNATNVVIKVCEFQFCNDPFLGVYYHKNNKSWMESEFRVYSSANNCTFEYVSQPFLMDLEGKQGNFKNLREFVFKNIDGYFKIYSKHTPINLVRDLPQGFSALEPLVDLPIGINITRFQTLLALHRSYLTPGDSSSGWTAGAAAYYVGYLQPRTFLLKYNENGTITDAVDCALDPLSETKCTLKSFTVEKGIYQTSNFRVQPTESIVRFPNITNLCPFGEVFNATRFASVYAWNRKRISNCVADYSVLYNSASFSTFKCYGVSPTKLNDLCFTNVYADSFVIRGDEVRQIAPGQTGKIADYNYKLPDDFTGCVIAWNSNNLDSKVGGNYNYLYRLFRKSNLKPFERDISTEIYQAGSTPCNGVEGFNCYFPLQSYGFQPTNGVGYQPYRVVVLSFELLHAPATVCGPKKSTNLVKNKCVNFGSGSGQYIKANSKFIGITELGSGSGYIPEAPRDGQAYVRKDGEWVLLSTFLGGSHHHHHH

SEQ ID NO: 43 - protein, 695 aa, Artificial Sequence
  NTD-RBD-ferritin
QCVNLTTRTQLPPAYTNSFTRGVYYPDKVFRSSVLHSTQDLFLPFFSNVTWFHAIHVSGTNGTKRFDNPVLPFNDGVYFASTEKSNIIRGWIFGTTLDSKTQSLLIVNNATNVVIKVCEFQFCNDPFLGVYYHKNNKSWMESEFRVYSSANNCTFEYVSQPFLMDLEGKQGNFKNLREFVFKNIDGYFKIYSKHTPINLVRDLPQGFSALEPLVDLPIGINITRFQTLLALHRSYLTPGDSSSGWTAGAAAYYVGYLQPRTFLLKYNENGTITDAVDCALDPLSETKCTLKSFTVEKGIYQTSNFRVQPTESIVRFPNITNLCPFGEVFNATRFASVYAWNRKRISNCVADYSVLYNSASFSTFKCYGVSPTKLNDLCFTNVYADSFVIRGDEVRQIAPGQTGKIADYNYKLPDDFTGCVIAWNSNNLDSKVGGNYNYLYRLFRKSNLKPFERDISTEIYQAGSTPCNGVEGFNCYFPLQSYGFQPTNGVGYQPYRVVVLSFELLHAPATVCGPKKSTNLVKNKCVNFMLSKDIIKLLNEQVNKEMNSSNLYMSMSSWCYTHSLDGAGLFLFDHAAEEYEHAKKLIIFLNENNVPVQLTSISAPEHKFEGLTQIFQKAYEHEQHISESINNIVDHAIKSKDHATFNFLQWYVAEQHEEEVLFKDILDKIELIGNENHGLYLADQYVKGIAKSRKS

SEQ ID NO: 44 - protein, 759 aa, Artificial Sequence
  NTD-RBD- HBsAg
QCVNLTTRTQLPPAYTNSFTRGVYYPDKVFRSSVLHSTQDLFLPFFSNVTWFHAIHVSGTNGTKRFDNPVLPFNDGVYFASTEKSNIIRGWIFGTTLDSKTQSLLIVNNATNVVIKVCEFQFCNDPFLGVYYHKNNKSWMESEFRVYSSANNCTFEYVSQPFLMDLEGKQGNFKNLREFVFKNIDGYFKIYSKHTPINLVRDLPQGFSALEPLVDLPIGINITRFQTLLALHRSYLTPGDSSSGWTAGAAAYYVGYLQPRTFLLKYNENGTITDAVDCALDPLSETKCTLKSFTVEKGIYQTSNFRVQPTESIVRFPNITNLCPFGEVFNATRFASVYAWNRKRISNCVADYSVLYNSASFSTFKCYGVSPTKLNDLCFTNVYADSFVIRGDEVRQIAPGQTGKIADYNYKLPDDFTGCVIAWNSNNLDSKVGGNYNYLYRLFRKSNLKPFERDISTEIYQAGSTPCNGVEGFNCYFPLQSYGFQPTNGVGYQPYRVVVLSFELLHAPATVCGPKKSTNLVKNKCVNFGSGSGMENITSGFLGPLLVLQAGFFLLTRILTIPQSLDSWWTSLNFLGGSPVCLGQNSQSPTSNHSPTSCPPICPGYRWMCLRRFIIFLFILLLCLIFLLVLLDYQGMLPVCPLIPGSTTTSTGPCKTCTTPAQGNSMFPSCCCTKPTDGNCTCIPIPSSWAFAKYLWEWASVRFSWLSLLVPFVQWFVGLSPTVWLSAIWMMWYWGPSLYSIVSPFIPLLPIFFCLWVYI

SEQ ID NO: 45 - DNA, 1500 bp, Artificial Sequence
  RBD-HBsAg-6*HIS
ggatccgccgccaccatgggcgtgcccgctgtgccagaggccagctctcctaggtggggcaccctgctgctggccatctttctggccgccagcagaggcctggtggccgctagagtgcagcctaccgagagcatcgtgcggttcccaaacatcaccaacctgtgtcctttcggcgaggtgttcaatgccaccaggttcgctagcgtgtatgcctggaacaggaagaggatctccaattgtgtggctgactactccgtgctgtacaacagcgcttcctttagcaccttcaagtgctacggcgtgtcccccaccaagctgaacgacttgtgctttaccaacgtgtatgccgacagctttgtgatcaggggcgacgaggtgcggcagattgctcctggacagaccggaaagatcgctgactataattacaagctgcccgacgacttcaccggctgcgttatcgcttggaatagcaacaatctggattccaaggtgggcggcaattacaattatctgtaccggctgttcaggaagtccaacctgaagcccttcgagagggatatcagcaccgagatctatcaggctggctccaccccctgtaacggcgttgaaggattcaattgctacttccccctgcagagctacggctttcagcctaccaatggcgtgggctatcagccctacagggtggttgtgctgagctttgagctgctgcacgctcctgctaccgtgtgtggaccaaagaagtccaccaacctggtgaagaataagtgcgtgaattttggatctggaagcggaatggagaacatcacctccggcttcctgggcccactgttggttctgcaggccggattcttcctgctgaccagaatcctgaccatcccccagtccctggacagctggtggacatctctgaattttctgggcggctcccccgtgtgcctgggacagaactctcagagccccaccagcaaccactccccaacaagctgcccccctatctgtcccggatataggtggatgtgtctgaggcggttcatcatcttcctgtttatcctgctgctgtgcctgatcttcctgctggtgctgctggactaccagggcatgctgccagtgtgccctctgatcccaggctctaccaccaccagcaccggaccttgtaagacctgcaccacccctgcccagggaaatagcatgtttccttcctgttgctgcaccaagcccaccgatggcaactgcacctgtatccccatccctagcagctgggcctttgctaagtacctgtgggagtgggcttccgtgcggtttagctggctgtccctgctggtgcctttcgtgcagtggttcgtgggcctgagccctacagtgtggctgtctgctatctggatgatgtggtattggggccctagcctgtacagcatcgtgtccccattcattcctctgctgcctatctttttctgcctgtgggtgtatatccaccaccaccaccatcactgactcgag

SEQ ID NO: 46 - DNA, 1644 bp, Artificial Sequence
  NTD-HBsAg-6*HIS
ggatccgccgccaccatgttcgtgtttctggtgctgctgcccctggtgtcctcccagtgtgttaatctgaccaccaggacccagctgcctcctgcttacaccaattcctttaccaggggcgtgtactaccccgacaaggtgttcaggtcctccgtgctgcacagcacccaggatctgttcctgcctttctttagcaacgtgacctggttccacgctatccacgtgagcggcaccaacggaaccaagagattcgacaatcccgtgctgcccttcaacgatggcgtgtacttcgccagcaccgagaagagcaacatcatccggggctggatcttcggcaccaccttggattccaagacccagagcctgctgatcgtgaacaacgctaccaacgtggtcattaaggtgtgtgagttccagttttgtaacgacccctttctgggcgtgtattatcacaagaacaataagtcctggatggagagcgagtttagggtgtattcctccgctaacaactgcacctttgagtatgtgagccagccttttctgatggacctggagggcaagcagggcaatttcaagaacctgagggagttcgtgtttaagaacatcgatggctactttaagatctactccaagcacacccctatcaacctggtgcgggatctgcctcagggctttagcgctctggagcctctggtggatctgccaatcggcatcaatatcacccggtttcagaccctgctggctctgcacaggagctacctgacccctggagatagctccagcggctggacagctggagctgctgcttactacgtgggctacctgcagcccagaacctttctgctgaagtacaatgagaacggcaccatcaccgacgccgtggattgcgctctggaccctttgtccgagaccaagtgtaccctgggatctggaagcggaatggagaacatcacctccggcttcctgggcccactgttggttctgcaggccggattcttcctgctgaccagaatcctgaccatcccccagtccctggacagctggtggacatctctgaattttctgggcggctcccccgtgtgcctgggacagaactctcagagccccaccagcaaccactccccaacaagctgcccccctatctgtcccggatataggtggatgtgtctgaggcggttcatcatcttcctgtttatcctgctgctgtgcctgatcttcctgctggtgctgctggactaccagggcatgctgccagtgtgccctctgatcccaggctctaccaccaccagcaccggaccttgtaagacctgcaccacccctgcccagggaaatagcatgtttccttcctgttgctgcaccaagcccaccgatggcaactgcacctgtatccccatccctagcagctgggcctttgctaagtacctgtgggagtgggcttccgtgcggtttagctggctgtccctgctggtgcctttcgtgcagtggttcgtgggcctgagccctacagtgtggctgtctgctatctggatgatgtggtattggggccctagcctgtacagcatcgtgtccccattcattcctctgctgcctatctttttctgcctgtgggtgtatatccaccaccaccaccatcactgactcgag

SEQ ID NO: 47 - DNA, 903 bp, Artificial Sequence
  RBD-foldon-6*HIS
ggatccgccgccaccatgggcgtgcccgctgtgccagaggccagctctcctaggtggggcaccctgctgctggccatctttctggccgccagcagaggcctggtggccgctagagtgcagcctaccgagagcatcgtgcggttcccaaacatcaccaacctgtgtcctttcggcgaggtgttcaatgccaccaggttcgctagcgtgtatgcctggaacaggaagaggatctccaattgtgtggctgactactccgtgctgtacaacagcgcttcctttagcaccttcaagtgctacggcgtgtcccccaccaagctgaacgacttgtgctttaccaacgtgtatgccgacagctttgtgatcaggggcgacgaggtgcggcagattgctcctggacagaccggaaagatcgctgactataattacaagctgcccgacgacttcaccggctgcgttatcgcttggaatagcaacaatctggattccaaggtgggcggcaattacaattatctgtaccggctgttcaggaagtccaacctgaagcccttcgagagggatatcagcaccgagatctatcaggctggctccaccccctgtaacggcgttgaaggattcaattgctacttccccctgcagagctacggctttcagcctaccaatggcgtgggctatcagccctacagggtggttgtgctgagctttgagctgctgcacgctcctgctaccgtgtgtggaccaaagaagtccaccaacctggtgaagaataagtgcgtgaattttggatctggatctggctacatccctgaggcccctagagatggccaggcttacgtgaggaaggacggcgaatgggtgctgctgagcaccttcctgggccatcaccaccaccaccattgactcgag

SEQ ID NO: 48 - DNA, 1047 bp, Artificial Sequence
  NTD-foldon-6*HIS
ggatccgccgccaccatgttcgtgtttctggtgctgctgcccctggtgtcctcccagtgtgttaatctgaccaccaggacccagctgcctcctgcttacaccaattcctttaccaggggcgtgtactaccccgacaaggtgttcaggtcctccgtgctgcacagcacccaggatctgttcctgcctttctttagcaacgtgacctggttccacgctatccacgtgagcggcaccaacggaaccaagagattcgacaatcccgtgctgcccttcaacgatggcgtgtacttcgccagcaccgagaagagcaacatcatccggggctggatcttcggcaccaccttggattccaagacccagagcctgctgatcgtgaacaacgctaccaacgtggtcattaaggtgtgtgagttccagttttgtaacgacccctttctgggcgtgtattatcacaagaacaataagtcctggatggagagcgagtttagggtgtattcctccgctaacaactgcacctttgagtatgtgagccagccttttctgatggacctggagggcaagcagggcaatttcaagaacctgagggagttcgtgtttaagaacatcgatggctactttaagatctactccaagcacacccctatcaacctggtgcgggatctgcctcagggctttagcgctctggagcctctggtggatctgccaatcggcatcaatatcacccggtttcagaccctgctggctctgcacaggagctacctgacccctggagatagctccagcggctggacagctggagctgctgcttactacgtgggctacctgcagcccagaacctttctgctgaagtacaatgagaacggcaccatcaccgacgccgtggattgcgctctggaccctttgtccgagaccaagtgtaccctgggatctggatctggctacatccctgaggcccctagagatggccaggcttacgtgaggaaggacggcgaatgggtgctgctgagcaccttcctgggccatcaccaccaccaccattgactcgag

SEQ ID NO: 49 - DNA, 1767 bp, Artificial Sequence
  NTD-RBD-foldon-8*HIS
ggatccgccgccaccatgttcgtgtttctggtgctgctgcccctggtgagctcccagtgtgttaacctgaccacccggacccagctgccacctgcttataccaacagctttacccggggcgtgtactaccctgacaaggtgttccggagctccgtgctgcacagcacacaggatctgtttctgcctttctttagcaacgtgacctggttccacgccatccacgtgagcggaaccaacggaaccaagcggttcgacaatcccgtgctgcctttcaacgatggcgtgtatttcgctagcaccgagaagagcaatatcatcaggggctggatcttcggcaccaccctggattccaagacccagtccctgctgatcgtgaataatgctaccaacgtggtcattaaggtgtgtgagttccagttttgtaacgacccctttctgggcgtgtattatcacaagaacaacaagtcctggatggagtccgagttccgggtgtactcctccgctaataattgcacctttgagtatgtgtcccagccttttctgatggacctggagggcaagcagggcaactttaagaacctgcgggagttcgtgtttaagaacatcgatggctatttcaagatctactccaagcacacccctatcaacctggtgagggacctgccccagggattttccgctctggagccactggtggacctgcctatcggaatcaacatcaccaggttccagaccctgctggctctgcacagatcctacctgacccctggcgattcctcctccggatggacagctggagctgctgcttactacgtgggctacctgcagcccaggaccttcttgctgaagtacaacgagaacggcaccatcaccgacgctgtggactgcgctctggaccctttgtccgagaccaagtgtaccctgaagagcttcaccgtggagaagggcatctatcagaccagcaacttccgggtgcagcccacagagagcatcgtgagattccctaacatcaccaacctgtgtcccttcggcgaggtgtttaatgccaccaggtttgctagcgtgtacgcttggaacaggaagcggatctccaattgcgtggccgattatagcgtgctgtacaactccgctagcttcagcacctttaagtgctatggcgtgagccctaccaagctgaatgatctgtgtttcaccaacgtgtatgctgactccttcgtgatccggggcgacgaagtgaggcagatcgctcctggacagaccggaaagatcgctgattataactacaagctgcccgacgactttaccggctgcgtgatcgcttggaatagcaataatctggactccaaggtgggcggcaattacaattatctgtataggctgttcaggaagtccaacctgaagcccttcgagagggatatctccaccgagatctatcaggctggctccaccccttgtaacggcgttgagggattcaactgttacttccccctgcagtcctacggctttcagcctaccaacggcgtgggctatcagccttaccgggtggttgtgctgtccttcgagctgctgcacgctcctgctaccgtgtgtggaccaaagaagtccaccaacctggtgaagaacaagtgtgtgaactttggatctggatctggctacatccctgaggcccctagagatggccaggcttacgtgaggaaggacggcgaatgggtgctgctgagcaccttcctgggccatcaccaccaccaccatcaccactgactcgag

SEQ ID NO: 50 - DNA, 3783 bp, Artificial Sequence
  S-foldon-8*HIS
ggatccgccgccaccatgttcgtgttcctggtgctgctgcccctggtgtctagccagtgtgtgaacctgaccaccaggacccagctgccaccagcttacaccaattccttcacccggggcgtgtactatcccgacaaggtgtttcggtccagcgtgctgcactccacccaggatctgtttctgccctttttctccaacgtgacctggttccacgccatccacgtgagcggaaccaacggaaccaagcggttcgataaccccgtgctgccctttaatgacggcgtgtactttgcttccaccgagaagtccaatatcatccggggctggatctttggcaccaccctggattccaagacccagtccctgctgatcgtgaataacgccaccaatgtggtcattaaggtgtgtgagtttcagttctgtaacgaccctttcctgggcgtgtattatcacaagaataacaagagctggatggagtccgagttccgggtgtactccagcgctaataactgcacctttgagtacgtgtcccagccctttctgatggatctggagggcaagcagggcaactttaagaacctgcgggagttcgtgtttaagaatatcgatggctattttaagatctacagcaagcacacccctatcaatctggtgagggacctgcctcagggcttctctgctctggagcctctggtggatctgcctatcggcatcaatatcacccggtttcagaccctgctggccctgcatagaagctatctgacccccggcgacagctcctctggatggacagctggagccgctgcttattacgtgggctatctgcagcccaggacctttctgctgaagtataatgagaacggcaccatcaccgatgctgtggactgtgccctggaccctctgtctgagaccaagtgcaccctgaagtcctttaccgtggagaagggcatctatcagacctccaacttccgggtgcagcccacagagagcatcgtgagattccctaatatcaccaatctgtgccctttcggcgaggtgttcaacgctaccaggtttgcctccgtgtatgcctggaatcggaagcggatctccaactgtgtggctgactattccgtgctgtataactccgcctccttcagcaccttcaagtgctatggcgtgagccctaccaagctgaacgacctgtgctttaccaacgtgtatgctgattccttcgtgatccggggcgacgaggtgagacagatcgctcctggacagaccggcaagatcgccgattataactacaagctgcctgatgatttcaccggctgtgtgatcgcttggaacagcaacaatctggatagcaaggtgggcggcaattacaactatctgtaccggctgtttcggaagagcaacctgaagcccttcgagagggatatctccaccgagatctatcaggccggcagcaccccttgcaatggcgttgaaggcttcaactgttatttccccctgcagagctatggctttcagcccaccaatggcgtgggctaccagccttaccgggtggttgtgctgagcttcgagctgctgcacgcccctgctacagtgtgtggaccaaagaagtccaccaacctggtgaagaataagtgcgtgaatttcaatttcaacggcctgaccggcaccggcgtgttgacagaaagcaacaagaagttcctgcccttccagcagtttggccgggatatcgctgacaccaccgatgctgtccgggaccctcagacactggagatcctggatatcaccccttgttcctttggcggcgtgtccgtgatcacccctggaacaaacacctccaatcaggtggccgtgctgtaccaggacgtgaactgtaccgaggtgcctgtggccatccacgctgatcagctgaccccaacctggagggtgtattccaccggctccaatgtgtttcagaccagggctggctgtctgatcggcgctgaacacgtgaacaactcctacgagtgtgatatccctatcggcgctggcatctgcgcctcttaccagacacagaccaatagccccaggagggccagatccgtggcttctcagagcatcatcgcctacaccatgagcctgggcgccgaaaattccgtggcttatagcaacaacagcatcgctatccctaccaatttcaccatcagcgtgaccaccgagatcctgcccgtgtctatgaccaagacctccgtggactgtaccatgtatatctgcggcgacagcaccgagtgcagcaacttgctgctgcagtatggcagcttctgcacccagctgaatagggctctgaccggcatcgctgtggagcaggataagaacacccaggaggtgttcgcccaggtgaagcagatctataagacccctcctatcaaggactttggcggcttcaacttcagccagatcctgcccgaccctagcaagccaagcaagaggtcctttatcgaggatctgctgtttaacaaggtgaccctggctgacgctggctttatcaagcagtatggcgattgtctgggcgatatcgccgccagagatctgatctgcgctcagaagttcaacggcctcaccgtgctgcctcctctgttgacagacgagatgatcgctcagtacacctccgccctgctggctggaacaatcacctccggatggaccttcggcgccggagctgctttgcagatcccattcgccatgcagatggcctaccggttcaacggcatcggcgtgacacagaatgtgctgtatgagaaccagaagctgatcgccaaccagttcaactccgccatcggcaagatccaggatagcctgagcagcaccgcctccgctttgggaaagctgcaggacgtggtgaatcagaacgcccaggccctgaacaccctggttaagcagctgtccagcaacttcggcgccatctcctccgtgctgaacgatatcctgtccaggctggacaaggtggaggccgaagtgcagatcgatcggctgatcaccggcaggctgcagtctttgcagacctatgtgacccagcagctgatccgggctgccgaaatcagagcctccgctaatctggccgctaccaagatgtccgagtgcgtgctgggccagtccaagagagtggatttctgcggcaagggctatcacctgatgagcttcccccagtccgctcctcacggagttgtgtttctgcacgtgacctacgtgcccgcccaggaaaagaactttaccaccgcccctgctatctgccacgacggaaaggctcactttcccagggagggcgtgttcgtgtccaacggaacccactggttcgtgacccagcggaacttttatgagccccagatcatcaccaccgataacacctttgtgtccggcaattgcgacgtggtcattggcatcgtgaataataccgtgtacgaccctctgcagcccgagttggactccttcaaggaggagctggacaagtacttcaagaatcacaccagccctgacgtggacctgggcgatatttccggcatcaacgccagcgtggtgaatatccagaaggagatcgacaggctgaacgaggtggctaagaatctgaacgagtccctgatcgacctgcaggagctgggaaagtacgagcagtacatcaagtggcctggatctggatctggctacatccctgaggcccctagagatggccaggcttacgtgaggaaggacggcgaatgggtgctgctgagcaccttcctgggccatcaccaccaccaccatcaccactgactcgag

SEQ ID NO: 51 - DNA, 867 bp, Artificial Sequence
  RBD-P2-6*HIS
ggatccgccgccaccatgggcgtgcccgctgtgccagaggccagctctcctaggtggggcaccctgctgctggccatctttctggccgccagcagaggcctggtggccgctagagtgcagcctaccgagagcatcgtgcggttcccaaacatcaccaacctgtgtcctttcggcgaggtgttcaatgccaccaggttcgctagcgtgtatgcctggaacaggaagaggatctccaattgtgtggctgactactccgtgctgtacaacagcgcttcctttagcaccttcaagtgctacggcgtgtcccccaccaagctgaacgacttgtgctttaccaacgtgtatgccgacagctttgtgatcaggggcgacgaggtgcggcagattgctcctggacagaccggaaagatcgctgactataattacaagctgcccgacgacttcaccggctgcgttatcgcttggaatagcaacaatctggattccaaggtgggcggcaattacaattatctgtaccggctgttcaggaagtccaacctgaagcccttcgagagggatatcagcaccgagatctatcaggctggctccaccccctgtaacggcgttgaaggattcaattgctacttccccctgcagagctacggctttcagcctaccaatggcgtgggctatcagccctacagggtggttgtgctgagctttgagctgctgcacgctcctgctaccgtgtgtggaccaaagaagtccaccaacctggtgaagaataagtgcgtgaattttggatctggaagcggacagtacatcaaggccaattccaagttcatcggcatcaccgagctgcaccaccaccaccatcactgactcgag

SEQ ID NO: 52 - DNA, 1014 bp, Artificial Sequence
  NTD- P2-6*HIS
ggatccgccgccaccatgttcgtgtttctggtgctgctgcccctggtgtcctcccagtgtgttaatctgaccaccaggacccagctgcctcctgcttacaccaattcctttaccaggggcgtgtactaccccgacaaggtgttcaggtcctccgtgctgcacagcacccaggatctgttcctgcctttctttagcaacgtgacctggttccacgctatccacgtgagcggcaccaacggaaccaagagattcgacaatcccgtgctgcccttcaacgatggcgtgtacttcgccagcaccgagaagagcaacatcatccggggctggatcttcggcaccaccttggattccaagacccagagcctgctgatcgtgaacaacgctaccaacgtggtcattaaggtgtgtgagttccagttttgtaacgacccctttctgggcgtgtattatcacaagaacaataagtcctggatggagagcgagtttagggtgtattcctccgctaacaactgcacctttgagtatgtgagccagccttttctgatggacctggagggcaagcagggcaatttcaagaacctgagggagttcgtgtttaagaacatcgatggctactttaagatctactccaagcacacccctatcaacctggtgcgggatctgcctcagggctttagcgctctggagcctctggtggatctgccaatcggcatcaatatcacccggtttcagaccctgctggctctgcacaggagctacctgacccctggagatagctccagcggctggacagctggagctgctgcttactacgtgggctacctgcagcccagaacctttctgctgaagtacaatgagaacggcaccatcaccgacgccgtggattgcgctctggaccctttgtccgagaccaagtgtaccctgggatctggaagcggacagtacatcaaggccaattccaagttcatcggcatcaccgagctgaaacaccaccaccaccatcactgactcgag

SEQ ID NO: 53 - DNA, 1731 bp, Artificial Sequence
  S1-P2-8*HIS
ggatccgccgccaccatgttcgtgtttctggtgctgctgcccctggtgagctcccagtgtgttaacctgaccacccggacccagctgccacctgcttataccaacagctttacccggggcgtgtactaccctgacaaggtgttccggagctccgtgctgcacagcacacaggatctgtttctgcctttctttagcaacgtgacctggttccacgccatccacgtgagcggaaccaacggaaccaagcggttcgacaatcccgtgctgcctttcaacgatggcgtgtatttcgctagcaccgagaagagcaatatcatcaggggctggatcttcggcaccaccctggattccaagacccagtccctgctgatcgtgaataatgctaccaacgtggtcattaaggtgtgtgagttccagttttgtaacgacccctttctgggcgtgtattatcacaagaacaacaagtcctggatggagtccgagttccgggtgtactcctccgctaataattgcacctttgagtatgtgtcccagccttttctgatggacctggagggcaagcagggcaactttaagaacctgcgggagttcgtgtttaagaacatcgatggctatttcaagatctactccaagcacacccctatcaacctggtgagggacctgccccagggattttccgctctggagccactggtggacctgcctatcggaatcaacatcaccaggttccagaccctgctggctctgcacagatcctacctgacccctggcgattcctcctccggatggacagctggagctgctgcttactacgtgggctacctgcagcccaggaccttcttgctgaagtacaacgagaacggcaccatcaccgacgctgtggactgcgctctggaccctttgtccgagaccaagtgtaccctgaagagcttcaccgtggagaagggcatctatcagaccagcaacttccgggtgcagcccacagagagcatcgtgagattccctaacatcaccaacctgtgtcccttcggcgaggtgtttaatgccaccaggtttgctagcgtgtacgcttggaacaggaagcggatctccaattgcgtggccgattatagcgtgctgtacaactccgctagcttcagcacctttaagtgctatggcgtgagccctaccaagctgaatgatctgtgtttcaccaacgtgtatgctgactccttcgtgatccggggcgacgaagtgaggcagatcgctcctggacagaccggaaagatcgctgattataactacaagctgcccgacgactttaccggctgcgtgatcgcttggaatagcaataatctggactccaaggtgggcggcaattacaattatctgtataggctgttcaggaagtccaacctgaagcccttcgagagggatatctccaccgagatctatcaggctggctccaccccttgtaacggcgttgagggattcaactgttacttccccctgcagtcctacggctttcagcctaccaacggcgtgggctatcagccttaccgggtggttgtgctgtccttcgagctgctgcacgctcctgctaccgtgtgtggaccaaagaagtccaccaacctggtgaagaacaagtgtgtgaactttggatctggaagcggacagtacatcaaggccaattccaagttcatcggcatcaccgagctgcaccaccaccaccatcaccaccactgactcgag

SEQ ID NO: 54 - DNA, 963 bp, Artificial Sequence
  RBD-P2-foldon-6*HIS
ggatccgccgccaccatgggcgtgcccgctgtgccagaggccagctctcctaggtggggcaccctgctgctggccatctttctggccgccagcagaggcctggtggccgctagagtgcagcctaccgagagcatcgtgcggttcccaaacatcaccaacctgtgtcctttcggcgaggtgttcaatgccaccaggttcgctagcgtgtatgcctggaacaggaagaggatctccaattgtgtggctgactactccgtgctgtacaacagcgcttcctttagcaccttcaagtgctacggcgtgtcccccaccaagctgaacgacttgtgctttaccaacgtgtatgccgacagctttgtgatcaggggcgacgaggtgcggcagattgctcctggacagaccggaaagatcgctgactataattacaagctgcccgacgacttcaccggctgcgttatcgcttggaatagcaacaatctggattccaaggtgggcggcaattacaattatctgtaccggctgttcaggaagtccaacctgaagcccttcgagagggatatcagcaccgagatctatcaggctggctccaccccctgtaacggcgttgaaggattcaattgctacttccccctgcagagctacggctttcagcctaccaatggcgtgggctatcagccctacagggtggttgtgctgagctttgagctgctgcacgctcctgctaccgtgtgtggaccaaagaagtccaccaacctggtgaagaataagtgcgtgaattttggatctggatctggccagtacatcaaggctaacagcaagtttatcggcatcaccgagctgggctccggctctggatatatccccgaggctcccagagacggccaggcttacgttaggaaggacggcgagtgggtgctgctgtctaccttcctgggccaccaccaccaccatcactgactcgag

SEQ ID NO: 55 - DNA, 1107 bp, Artificial Sequence
  NTD-P2-foldon-6*HIS
ggatccgccgccaccatgttcgtgtttctggtgctgctgcccctggtgtcctcccagtgtgttaatctgaccaccaggacccagctgcctcctgcttacaccaattcctttaccaggggcgtgtactaccccgacaaggtgttcaggtcctccgtgctgcacagcacccaggatctgttcctgcctttctttagcaacgtgacctggttccacgctatccacgtgagcggcaccaacggaaccaagagattcgacaatcccgtgctgcccttcaacgatggcgtgtacttcgccagcaccgagaagagcaacatcatccggggctggatcttcggcaccaccttggattccaagacccagagcctgctgatcgtgaacaacgctaccaacgtggtcattaaggtgtgtgagttccagttttgtaacgacccctttctgggcgtgtattatcacaagaacaataagtcctggatggagagcgagtttagggtgtattcctccgctaacaactgcacctttgagtatgtgagccagccttttctgatggacctggagggcaagcagggcaatttcaagaacctgagggagttcgtgtttaagaacatcgatggctactttaagatctactccaagcacacccctatcaacctggtgcgggatctgcctcagggctttagcgctctggagcctctggtggatctgccaatcggcatcaatatcacccggtttcagaccctgctggctctgcacaggagctacctgacccctggagatagctccagcggctggacagctggagctgctgcttactacgtgggctacctgcagcccagaacctttctgctgaagtacaatgagaacggcaccatcaccgacgccgtggattgcgctctggaccctttgtccgagaccaagtgtaccctgggatctggatctggccagtacatcaaggctaacagcaagtttatcggcatcaccgagctgggctccggctctggatatatccccgaggctcccagagacggccaggcttacgttaggaaggacggcgagtgggtgctgctgtctaccttcctgggccaccaccaccaccatcactgactcgag

SEQ ID NO: 56 - DNA, 1827 bp, Artificial Sequence
  S1-P2-foldon-6*HIS
ggatccgccgccaccatgttcgtgtttctggtgctgctgcccctggtgagctcccagtgtgttaacctgaccacccggacccagctgccacctgcttataccaacagctttacccggggcgtgtactaccctgacaaggtgttccggagctccgtgctgcacagcacacaggatctgtttctgcctttctttagcaacgtgacctggttccacgccatccacgtgagcggaaccaacggaaccaagcggttcgacaatcccgtgctgcctttcaacgatggcgtgtatttcgctagcaccgagaagagcaatatcatcaggggctggatcttcggcaccaccctggattccaagacccagtccctgctgatcgtgaataatgctaccaacgtggtcattaaggtgtgtgagttccagttttgtaacgacccctttctgggcgtgtattatcacaagaacaacaagtcctggatggagtccgagttccgggtgtactcctccgctaataattgcacctttgagtatgtgtcccagccttttctgatggacctggagggcaagcagggcaactttaagaacctgcgggagttcgtgtttaagaacatcgatggctatttcaagatctactccaagcacacccctatcaacctggtgagggacctgccccagggattttccgctctggagccactggtggacctgcctatcggaatcaacatcaccaggttccagaccctgctggctctgcacagatcctacctgacccctggcgattcctcctccggatggacagctggagctgctgcttactacgtgggctacctgcagcccaggaccttcttgctgaagtacaacgagaacggcaccatcaccgacgctgtggactgcgctctggaccctttgtccgagaccaagtgtaccctgaagagcttcaccgtggagaagggcatctatcagaccagcaacttccgggtgcagcccacagagagcatcgtgagattccctaacatcaccaacctgtgtcccttcggcgaggtgtttaatgccaccaggtttgctagcgtgtacgcttggaacaggaagcggatctccaattgcgtggccgattatagcgtgctgtacaactccgctagcttcagcacctttaagtgctatggcgtgagccctaccaagctgaatgatctgtgtttcaccaacgtgtatgctgactccttcgtgatccggggcgacgaagtgaggcagatcgctcctggacagaccggaaagatcgctgattataactacaagctgcccgacgactttaccggctgcgtgatcgcttggaatagcaataatctggactccaaggtgggcggcaattacaattatctgtataggctgttcaggaagtccaacctgaagcccttcgagagggatatctccaccgagatctatcaggctggctccaccccttgtaacggcgttgagggattcaactgttacttccccctgcagtcctacggctttcagcctaccaacggcgtgggctatcagccttaccgggtggttgtgctgtccttcgagctgctgcacgctcctgctaccgtgtgtggaccaaagaagtccaccaacctggtgaagaacaagtgtgtgaactttggatctggatctggccagtacatcaaggctaacagcaagtttatcggcatcaccgagctgggctccggctctggatatatccccgaggctcccagagacggccaggcttacgttaggaaggacggcgagtgggtgctgctgtctaccttcctgggccaccaccaccaccatcaccaccactgactcgag

SEQ ID NO: 57 - DNA, 1371 bp, Artificial Sequence
  RBD-ferritin  LC-6*HIS
ggatccgccgccaccatgggcgtgcccgctgtgccagaggccagctctcctaggtggggcaccctgctgctggccatctttctggccgccagcagaggcctggtggccgctagagtgcagcctaccgagagcatcgtgcggttcccaaacatcaccaacctgtgtcctttcggcgaggtgttcaatgccaccaggttcgctagcgtgtatgcctggaacaggaagaggatctccaattgtgtggctgactactccgtgctgtacaacagcgcttcctttagcaccttcaagtgctacggcgtgtcccccaccaagctgaacgacttgtgctttaccaacgtgtatgccgacagctttgtgatcaggggcgacgaggtgcggcagattgctcctggacagaccggaaagatcgctgactataattacaagctgcccgacgacttcaccggctgcgttatcgcttggaatagcaacaatctggattccaaggtgggcggcaattacaattatctgtaccggctgttcaggaagtccaacctgaagcccttcgagagggatatcagcaccgagatctatcaggctggctccaccccctgtaacggcgttgaaggattcaattgctacttccccctgcagagctacggctttcagcctaccaatggcgtgggctatcagccctacagggtggttgtgctgagctttgagctgctgcacgctcctgctaccgtgtgtggaccaaagaagtccaccaacctggtgaagaataagtgcgtgaattttggatctggatctggcgagtacggcagccacggaaacgtggctaccgagttgcaggcctatgctaagctgcacctggagaggtcctatgactacctgctgtccgccgcttattttaacaactaccagaccaacagggccggcttttccaagctgtttaagaagctgagcgacgaggcctggagcaagaccatcgatatcatcaagcacgtgaccaagcggggcgataagatgaattttgaccagcacagcaccatgaagaccgagcggaagaactataccgctgagaatcacgagctggaggccctggctaaggctttggatacccagaaggagctggctgagcgggctttctatatccacagggaggctacccggaatagccagcacctgcacgaccctgagatcgctcagtacctggaggaggagttcatcgaggatcacgctgagaagatccggaccctggccggacataccagcgatttgaagaagttcatcaccgccaataatggccacgacctgagcctggctctgtacgttttcgacgagtacctgcagaagaccgtgcaccaccaccatcaccactgactcgag

SEQ ID NO: 58 - DNA, 1347 bp, Artificial Sequence
  RBD-ferritin HC-FLAG
ggatccgccgccaccatgggcgtgcccgctgtgccagaggccagctctcctaggtggggcaccctgctgctggccatctttctggccgccagcagaggcctggtggccgctagagtgcagcctaccgagagcatcgtgcggttcccaaacatcaccaacctgtgtcctttcggcgaggtgttcaatgccaccaggttcgctagcgtgtatgcctggaacaggaagaggatctccaattgtgtggctgactactccgtgctgtacaacagcgcttcctttagcaccttcaagtgctacggcgtgtcccccaccaagctgaacgacttgtgctttaccaacgtgtatgccgacagctttgtgatcaggggcgacgaggtgcggcagattgctcctggacagaccggaaagatcgctgactataattacaagctgcccgacgacttcaccggctgcgttatcgcttggaatagcaacaatctggattccaaggtgggcggcaattacaattatctgtaccggctgttcaggaagtccaacctgaagcccttcgagagggatatcagcaccgagatctatcaggctggctccaccccctgtaacggcgttgaaggattcaattgctacttccccctgcagagctacggctttcagcctaccaatggcgtgggctatcagccctacagggtggttgtgctgagctttgagctgctgcacgctcctgctaccgtgtgtggaccaaagaagtccaccaacctggtgaagaataagtgcgtgaattttggatctggatctggcagatcctgccggaactccatgcggcagcagatccagatggaggtgggcgcttccctgcagtacctggctatgggagcccactttagcaaggatgtggtgaacaggcccggctttgcccagttgtttttcgacgccgcttccgaggagagggagcatgctatgaagctgatcgagtacctgctgatgcggggcgagctgacaaacgacgtgagctctctgctgcaggtgcggcctcctacaagatccagctggaagggcggcgtggaggctttggaacacgctttgagcatggagagcgatgtgaccaagagcatcaggaatgtgatcaaggcctgtgaggatgacagcgagtttaatgattatcacctggtggattacctgaccggcgattttctggaggagcagtacaagggccagagggacctggctggaaaggcttctaccctgaagaagctgatggaccggcacgaggctctgggagaattcatcttcgataagaagctgctgggcatcgacgtggattataaggatgatgacgataagtgactcgag

SEQ ID NO: 59 - DNA, 1374 bp, Artificial Sequence
  RBD194-HBsAg
ggatccgccgccaccatggagactgggctgcgctggcttctcctggtcgctgtgctcaaaggtgtccagtgtaacatcaccaacctgtgtcctttcggcgaggtgttcaatgccaccaggttcgctagcgtgtatgcctggaacaggaagaggatctccaattgtgtggctgactactccgtgctgtacaacagcgcttcctttagcaccttcaagtgctacggcgtgtcccccaccaagctgaacgacttgtgctttaccaacgtgtatgccgacagctttgtgatcaggggcgacgaggtgcggcagattgctcctggacagaccggaaagatcgctgactataattacaagctgcccgacgacttcaccggctgcgttatcgcttggaatagcaacaatctggattccaaggtgggcggcaattacaattatctgtaccggctgttcaggaagtccaacctgaagcccttcgagagggatatcagcaccgagatctatcaggctggctccaccccctgtaacggcgttgaaggattcaattgctacttccccctgcagagctacggctttcagcctaccaatggcgtgggctatcagccctacagggtggttgtgctgagctttgagctgctgcacgctcctgctaccgtgggatctggaagcggaatggagaacatcacctccggcttcctgggcccactgttggttctgcaggccggattcttcctgctgaccagaatcctgaccatcccccagtccctggacagctggtggacatctctgaattttctgggcggctcccccgtgtgcctgggacagaactctcagagccccaccagcaaccactccccaacaagctgcccccctatctgtcccggatataggtggatgtgtctgaggcggttcatcatcttcctgtttatcctgctgctgtgcctgatcttcctgctggtgctgctggactaccagggcatgctgccagtgtgccctctgatcccaggctctaccaccaccagcaccggaccttgtaagacctgcaccacccctgcccagggaaatagcatgtttccttcctgttgctgcaccaagcccaccgatggcaactgcacctgtatccccatccctagcagctgggcctttgctaagtacctgtgggagtgggcttccgtgcggtttagctggctgtccctgctggtgcctttcgtgcagtggttcgtgggcctgagccctacagtgtggctgtctgctatctggatgatgtggtattggggccctagcctgtacagcatcgtgtccccattcattcctctgctgcctatctttttctgcctgtgggtgtatatccaccaccaccaccatcactgactcgag

SEQ ID NO: 60 - DNA, 1491 bp, Artificial Sequence
  NTD-ferritin HC nucleotide sequence
ggatccgccgccaccatgttcgtgtttctggtgctgctgcccctggtgtcctcccagtgtgttaatctgaccaccaggacccagctgcctcctgcttacaccaattcctttaccaggggcgtgtactaccccgacaaggtgttcaggtcctccgtgctgcacagcacccaggatctgttcctgcctttctttagcaacgtgacctggttccacgctatccacgtgagcggcaccaacggaaccaagagattcgacaatcccgtgctgcccttcaacgatggcgtgtacttcgccagcaccgagaagagcaacatcatccggggctggatcttcggcaccaccttggattccaagacccagagcctgctgatcgtgaacaacgctaccaacgtggtcattaaggtgtgtgagttccagttttgtaacgacccctttctgggcgtgtattatcacaagaacaataagtcctggatggagagcgagtttagggtgtattcctccgctaacaactgcacctttgagtatgtgagccagccttttctgatggacctggagggcaagcagggcaatttcaagaacctgagggagttcgtgtttaagaacatcgatggctactttaagatctactccaagcacacccctatcaacctggtgcgggatctgcctcagggctttagcgctctggagcctctggtggatctgccaatcggcatcaatatcacccggtttcagaccctgctggctctgcacaggagctacctgacccctggagatagctccagcggctggacagctggagctgctgcttactacgtgggctacctgcagcccagaacctttctgctgaagtacaatgagaacggcaccatcaccgacgccgtggattgcgctctggaccctttgtccgagaccaagtgtaccctgggatctggatctggcagatcctgccggaactccatgcggcagcagatccagatggaggtgggcgcttccctgcagtacctggctatgggagcccactttagcaaggatgtggtgaacaggcccggctttgcccagttgtttttcgacgccgcttccgaggagagggagcatgctatgaagctgatcgagtacctgctgatgcggggcgagctgacaaacgacgtgagctctctgctgcaggtgcggcctcctacaagatccagctggaagggcggcgtggaggctttggaacacgctttgagcatggagagcgatgtgaccaagagcatcaggaatgtgatcaaggcctgtgaggatgacagcgagtttaatgattatcacctggtggattacctgaccggcgattttctggaggagcagtacaagggccagagggacctggctggaaaggcttctaccctgaagaagctgatggaccggcacgaggctctgggagaattcatcttcgataagaagctgctgggcatcgacgtggattataaggatgatgacgataagtgactcgag

SEQ ID NO: 61 - DNA, 1515 bp, Artificial Sequence
  NTD-ferritin  LC nucleotide sequence
ggatccgccgccaccatgttcgtgtttctggtgctgctgcccctggtgtcctcccagtgtgttaatctgaccaccaggacccagctgcctcctgcttacaccaattcctttaccaggggcgtgtactaccccgacaaggtgttcaggtcctccgtgctgcacagcacccaggatctgttcctgcctttctttagcaacgtgacctggttccacgctatccacgtgagcggcaccaacggaaccaagagattcgacaatcccgtgctgcccttcaacgatggcgtgtacttcgccagcaccgagaagagcaacatcatccggggctggatcttcggcaccaccttggattccaagacccagagcctgctgatcgtgaacaacgctaccaacgtggtcattaaggtgtgtgagttccagttttgtaacgacccctttctgggcgtgtattatcacaagaacaataagtcctggatggagagcgagtttagggtgtattcctccgctaacaactgcacctttgagtatgtgagccagccttttctgatggacctggagggcaagcagggcaatttcaagaacctgagggagttcgtgtttaagaacatcgatggctactttaagatctactccaagcacacccctatcaacctggtgcgggatctgcctcagggctttagcgctctggagcctctggtggatctgccaatcggcatcaatatcacccggtttcagaccctgctggctctgcacaggagctacctgacccctggagatagctccagcggctggacagctggagctgctgcttactacgtgggctacctgcagcccagaacctttctgctgaagtacaatgagaacggcaccatcaccgacgccgtggattgcgctctggaccctttgtccgagaccaagtgtaccctgggatctggatctggcgagtacggcagccacggaaacgtggctaccgagttgcaggcctatgctaagctgcacctggagaggtcctatgactacctgctgtccgccgcttattttaacaactaccagaccaacagggccggcttttccaagctgtttaagaagctgagcgacgaggcctggagcaagaccatcgatatcatcaagcacgtgaccaagcggggcgataagatgaattttgaccagcacagcaccatgaagaccgagcggaagaactataccgctgagaatcacgagctggaggccctggctaaggctttggatacccagaaggagctggctgagcgggctttctatatccacagggaggctacccggaatagccagcacctgcacgaccctgagatcgctcagtacctggaggaggagttcatcgaggatcacgctgagaagatccggaccctggccggacataccagcgatttgaagaagttcatcaccgccaataatggccacgacctgagcctggctctgtacgttttcgacgagtacctgcagaagaccgtgcaccaccaccatcaccactgactcgag

SEQ ID NO: 62 - DNA, 1455 bp, Artificial Sequence
  NTD-ferritin nucleotide sequence
ggatccgccgccaccatgttcgtgtttctggtgctgctgcccctggtgtcctcccagtgtgttaatctgaccaccaggacccagctgcctcctgcttacaccaattcctttaccaggggcgtgtactaccccgacaaggtgttcaggtcctccgtgctgcacagcacccaggatctgttcctgcctttctttagcaacgtgacctggttccacgctatccacgtgagcggcaccaacggaaccaagagattcgacaatcccgtgctgcccttcaacgatggcgtgtacttcgccagcaccgagaagagcaacatcatccggggctggatcttcggcaccaccttggattccaagacccagagcctgctgatcgtgaacaacgctaccaacgtggtcattaaggtgtgtgagttccagttttgtaacgacccctttctgggcgtgtattatcacaagaacaataagtcctggatggagagcgagtttagggtgtattcctccgctaacaactgcacctttgagtatgtgagccagccttttctgatggacctggagggcaagcagggcaatttcaagaacctgagggagttcgtgtttaagaacatcgatggctactttaagatctactccaagcacacccctatcaacctggtgcgggatctgcctcagggctttagcgctctggagcctctggtggatctgccaatcggcatcaatatcacccggtttcagaccctgctggctctgcacaggagctacctgacccctggagatagctccagcggctggacagctggagctgctgcttactacgtgggctacctgcagcccagaacctttctgctgaagtacaatgagaacggcaccatcaccgacgccgtggattgcgctctggaccctttgtccgagaccaagtgtaccctgggatctggatctggcgatatcatcaagctgctgaacgagcaggtgaataaggagatgaactcctccaacctgtacatgagcatgtccagctggtgttacacccactccctggacggcgctggattgtttctgttcgaccacgctgccgaggagtacgagcacgctaagaagctgatcatcttcctgaatgagaataatgtgcccgtgcagctgacctccatctccgctcctgagcacaagtttgagggcctgacccagatcttccagaaggcttacgagcacgagcagcacatcagcgagagcatcaacaacatcgtggaccacgctatcaagtccaaggaccacgccacctttaatttcctgcagtggtatgtggctgagcagcacgaggaggaggtgttgtttaaggatatcctggacaagatcgagctgatcggcaatgagaatcacggcctgtatctggctgaccagtatgtgaagggcatcgccaagagcaggaagagccaccaccaccaccatcactgactcgag

SEQ ID NO: 63 - DNA, 1311 bp, Artificial Sequence
  RBD-ferritin nucleotide sequence
ggatccgccgccaccatgggcgtgcccgctgtgccagaggccagctctcctaggtggggcaccctgctgctggccatctttctggccgccagcagaggcctggtggccgctagagtgcagcctaccgagagcatcgtgcggttcccaaacatcaccaacctgtgtcctttcggcgaggtgttcaatgccaccaggttcgctagcgtgtatgcctggaacaggaagaggatctccaattgtgtggctgactactccgtgctgtacaacagcgcttcctttagcaccttcaagtgctacggcgtgtcccccaccaagctgaacgacttgtgctttaccaacgtgtatgccgacagctttgtgatcaggggcgacgaggtgcggcagattgctcctggacagaccggaaagatcgctgactataattacaagctgcccgacgacttcaccggctgcgttatcgcttggaatagcaacaatctggattccaaggtgggcggcaattacaattatctgtaccggctgttcaggaagtccaacctgaagcccttcgagagggatatcagcaccgagatctatcaggctggctccaccccctgtaacggcgttgaaggattcaattgctacttccccctgcagagctacggctttcagcctaccaatggcgtgggctatcagccctacagggtggttgtgctgagctttgagctgctgcacgctcctgctaccgtgtgtggaccaaagaagtccaccaacctggtgaagaataagtgcgtgaattttggatctggatctggcgatatcatcaagctgctgaacgagcaggtgaataaggagatgaactcctccaacctgtacatgagcatgtccagctggtgttacacccactccctggacggcgctggattgtttctgttcgaccacgctgccgaggagtacgagcacgctaagaagctgatcatcttcctgaatgagaataatgtgcccgtgcagctgacctccatctccgctcctgagcacaagtttgagggcctgacccagatcttccagaaggcttacgagcacgagcagcacatcagcgagagcatcaacaacatcgtggaccacgctatcaagtccaaggaccacgccacctttaatttcctgcagtggtatgtggctgagcagcacgaggaggaggtgttgtttaaggatatcctggacaagatcgagctgatcggcaatgagaatcacggcctgtatctggctgaccagtatgtgaagggcatcgccaagagcaggaagagccaccaccaccaccatcactgactcgag

SEQ ID NO: 64 - protein, 15 aa, Artificial Sequence
  P2_1
QYIKANSKFIGITEL

SEQ ID NO: 65 - protein, 16 aa, Artificial Sequence
  P2_2
QYIKANSKFIGITELK

SEQ ID NO: 66 - protein, 16 aa, Artificial Sequence
  P2_3
MQYIKANSKFIGITEL

SEQ ID NO: 67 - protein, 27 aa, Artificial Sequence
  foldon_1
PEAPRDGQAYVRKDGEWVLLSTFLSPA

SEQ ID NO: 68 - protein, 27 aa, Artificial Sequence
  foldon_2
AGYIPEAPRDGQAYVRKDGEWVLLSTF

SEQ ID NO: 69 - protein, 27 aa, Artificial Sequence
  foldon_3
YIPEAPRDGQAYVRKDGEWVLLSTFLG

SEQ ID NO: 70 - protein, 173 aa, Artificial Sequence
  ferritin HC
RSCRNSMRQQIQMEVGASLQYLAMGAHFSKDVVNRPGFAQLFFDAASEEREHAMKLIEYLLMRGELTNDVSSLLQVRPPTRSSWKGGVEALEHALSMESDVTKSIRNVIKACEDDSEFNDYHLVDYLTGDFLEEQYKGQRDLAGKASTLKKLMDRHEALGEFIFDKKLLGIDV

SEQ ID NO: 71 - protein, 183 aa, Artificial Sequence
  ferritin LC
EYGSHGNVATELQAYAKLHLERSYDYLLSAAYFNNYQTNRAGFSKLFKKLSDEAWSKTIDIIKHVTKRGDKMNFDQHSTMKTERKNYTAENHELEALAKALDTQKELAERAFYIHREATRNSQHLHDPEIAQYLEEEFIEDHAEKIRTLAGHTSDLKKFITANNGHDLSLALYVFDEYLQKTV

SEQ ID NO: 72 - protein, 167 aa, Artificial Sequence
  Helicobacter pylori ferritin
MLSKDIIKLLNEQVNKEMNSSNLYMSMSSWCYTHSLDGAGLFLFDHAAEEYEHAKKLIIFLNENNVPVQLTSISAPEHKFEGLTQIFQKAYEHEQHISESINNIVDHAIKSKDHATFNFLQWYVAEQHEEEVLFKDILDKIELIGNENHGLYLADQYVKGIAKSRKS

SEQ ID NO: 73 - protein, 226 aa, Artificial Sequence
  HBsAg
MENITSGFLGPLLVLQAGFFLLTRILTIPQSLDSWWTSLNFLGGSPVCLGQNSQSPTSNHSPTSCPPICPGYRWMCLRRFIIFLFILLLCLIFLLVLLDYQGMLPVCPLIPGSTTTSTGPCKTCTTPAQGNSMFPSCCCTKPTDGNCTCIPIPSSWAFAKYLWEWASVRFSWLSLLVPFVQWFVGLSPTVWLSAIWMMWYWGPSLYSIVSPFIPLLPIFFCLWVYI

SEQ ID NO: 74 - protein, 32 aa, Artificial Sequence
  signal peptide_1
MGVPAVPEASSPRWGTLLLAIFLAASRGLVAA

SEQ ID NO: 75 - protein, 12 aa, Artificial Sequence
  signal peptide_2
MFVFLVLLPLVS

SEQ ID NO: 76 - protein, 223 aa, Artificial Sequence
  RBD Beta variant
RVQPTESIVRFPNITNLCPFGEVFNATRFASVYAWNRKRISNCVADYSVLYNSASFSTFKCYGVSPTKLNDLCFTNVYADSFVIRGDEVRQIAPGQTGNIADYNYKLPDDFTGCVIAWNSNNLDSKVGGNYNYLYRLFRKSNLKPFERDISTEIYQAGSTPCNGVKGFNCYFPLQSYGFQPTYGVGYQPYRVVVLSFELLHAPATVCGPKKSTNLVKNKCVNF

SEQ ID NO: 77 - protein, 288 aa, Artificial Sequence
  NTD Beta variant
QCVNFTTRTQLPPAYTNSFTRGVYYPDKVFRSSVLHSTQDLFLPFFSNVTWFHAIHVSGTNGTKRFANPVLPFNDGVYFASTEKSNIIRGWIFGTTLDSKTQSLLIVNNATNVVIKVCEFQFCNDPFLGVYYHKNNKSWMESEFRVYSSANNCTFEYVSQPFLMDLEGKQGNFKNLREFVFKNIDGYFKIYSKHTPINLVRGLPQGFSALEPLVDLPIGINITRFQTLHISYLTPGDSSSGWTAGAAAYYVGYLQPRTFLLKYNENGTITDAVDCALDPLSETKCTLK

SEQ ID NO: 78 - protein, 26 aa, Artificial Sequence
  foldon(bacteriophage T4 fibritinC)
YIPEAPRDGQAYVRKDGEWVLLSTFL

SEQ ID NO: 79 - protein, 557 aa, Artificial Sequence
  RBD-NTD-foldon(Beta variant)
QCVNFTTRTQLPPAYTNSFTRGVYYPDKVFRSSVLHSTQDLFLPFFSNVTWFHAIHVSGTNGTKRFANPVLPFNDGVYFASTEKSNIIRGWIFGTTLDSKTQSLLIVNNATNVVIKVCEFQFCNDPFLGVYYHKNNKSWMESEFRVYSSANNCTFEYVSQPFLMDLEGKQGNFKNLREFVFKNIDGYFKIYSKHTPINLVRGLPQGFSALEPLVDLPIGINITRFQTLHISYLTPGDSSSGWTAGAAAYYVGYLQPRTFLLKYNENGTITDAVDCALDPLSETKCTLKSFTVEKGIYQTSNFRVQPTESIVRFPNITNLCPFGEVFNATRFASVYAWNRKRISNCVADYSVLYNSASFSTFKCYGVSPTKLNDLCFTNVYADSFVIRGDEVRQIAPGQTGNIADYNYKLPDDFTGCVIAWNSNNLDSKVGGNYNYLYRLFRKSNLKPFERDISTEIYQAGSTPCNGVKGFNCYFPLQSYGFQPTYGVGYQPYRVVVLSFELLHAPATVCGPKKSTNLVKNKCVNFGSGSGYIPEAPRDGQAYVRKDGEWVLLSTFLG

SEQ ID NO: 80 - protein, 255 aa, Artificial Sequence
  RBD-foldon Beta variant
RVQPTESIVRFPNITNLCPFGEVFNATRFASVYAWNRKRISNCVADYSVLYNSASFSTFKCYGVSPTKLNDLCFTNVYADSFVIRGDEVRQIAPGQTGNIADYNYKLPDDFTGCVIAWNSNNLDSKVGGNYNYLYRLFRKSNLKPFERDISTEIYQAGSTPCNGVKGFNCYFPLQSYGFQPTYGVGYQPYRVVVLSFELLHAPATVCGPKKSTNLVKNKCVNFGSGSGYIPEAPRDGQAYVRKDGEWVLLSTFLG

SEQ ID NO: 81 - protein, 320 aa, Artificial Sequence
  NTD-foldon Beta variant
QCVNFTTRTQLPPAYTNSFTRGVYYPDKVFRSSVLHSTQDLFLPFFSNVTWFHAIHVSGTNGTKRFANPVLPFNDGVYFASTEKSNIIRGWIFGTTLDSKTQSLLIVNNATNVVIKVCEFQFCNDPFLGVYYHKNNKSWMESEFRVYSSANNCTFEYVSQPFLMDLEGKQGNFKNLREFVFKNIDGYFKIYSKHTPINLVRGLPQGFSALEPLVDLPIGINITRFQTLHISYLTPGDSSSGWTAGAAAYYVGYLQPRTFLLKYNENGTITDAVDCALDPLSETKCTLKGSGSGYIPEAPRDGQAYVRKDGEWVLLSTFLG

SEQ ID NO: 82 - protein, 1270 aa, Artificial Sequence
  Beta501Y.V2 Surface glycoprotein
MFVFLVLLPLVSSQCVNFTTRTQLPPAYTNSFTRGVYYPDKVFRSSVLHSTQDLFLPFFSNVTWFHAIHVSGTNGTKRFANPVLPFNDGVYFASTEKSNIIRGWIFGTTLDSKTQSLLIVNNATNVVIKVCEFQFCNDPFLGVYYHKNNKSWMESEFRVYSSANNCTFEYVSQPFLMDLEGKQGNFKNLREFVFKNIDGYFKIYSKHTPINLVRGLPQGFSALEPLVDLPIGINITRFQTLHISYLTPGDSSSGWTAGAAAYYVGYLQPRTFLLKYNENGTITDAVDCALDPLSETKCTLKSFTVEKGIYQTSNFRVQPTESIVRFPNITNLCPFGEVFNATRFASVYAWNRKRISNCVADYSVLYNSASFSTFKCYGVSPTKLNDLCFTNVYADSFVIRGDEVRQIAPGQTGNIADYNYKLPDDFTGCVIAWNSNNLDSKVGGNYNYLYRLFRKSNLKPFERDISTEIYQAGSTPCNGVKGFNCYFPLQSYGFQPTYGVGYQPYRVVVLSFELLHAPATVCGPKKSTNLVKNKCVNFNFNGLTGTGVLTESNKKFLPFQQFGRDIADTTDAVRDPQTLEILDITPCSFGGVSVITPGTNTSNQVAVLYQGVNCTEVPVAIHADQLTPTWRVYSTGSNVFQTRAGCLIGAEHVNNSYECDIPIGAGICASYQTQTNSPRRARSVASQSIIAYTMSLGVENSVAYSNNSIAIPTNFTISVTTEILPVSMTKTSVDCTMYICGDSTECSNLLLQYGSFCTQLNRALTGIAVEQDKNTQEVFAQVKQIYKTPPIKDFGGFNFSQILPDPSKPSKRSFIEDLLFNKVTLADAGFIKQYGDCLGDIAARDLICAQKFNGLTVLPPLLTDEMIAQYTSALLAGTITSGWTFGAGAALQIPFAMQMAYRFNGIGVTQNVLYENQKLIANQFNSAIGKIQDSLSSTASALGKLQDVVNQNAQALNTLVKQLSSNFGAISSVLNDILSRLDKVEAEVQIDRLITGRLQSLQTYVTQQLIRAAEIRASANLAATKMSECVLGQSKRVDFCGKGYHLMSFPQSAPHGVVFLHVTYVPAQEKNFTTAPAICHDGKAHFPREGVFVSNGTHWFVTQRNFYEPQIITTDNTFVSGNCDVVIGIVNNTVYDPLQPELDSFKEELDKYFKNHTSPDVDLGDISGINASVVNIQKEIDRLNEVAKNLNESLIDLQELGKYEQYIKWPWYIWLGFIAGLIAIVMVTIMLCCMTSCCSCLKGCCSCGSCCKFDEDDSEPVLKGVKLHYT

SEQ ID NO: 83 - protein, 223 aa, Artificial Sequence
  RBD Gamma variant
RVQPTESIVRFPNITNLCPFGEVFNATRFASVYAWNRKRISNCVADYSVLYNSASFSTFKCYGVSPTKLNDLCFTNVYADSFVIRGDEVRQIAPGQTGTIADYNYKLPDDFTGCVIAWNSNNLDSKVGGNYNYLYRLFRKSNLKPFERDISTEIYQAGSTPCNGVKGFNCYFPLQSYGFQPTYGVGYQPYRVVVLSFELLHAPATVCGPKKSTNLVKNKCVNF

SEQ ID NO: 84 - protein, 291 aa, Artificial Sequence
  NTD Gamma variant
QCVNFTNRTQLPSAYTNSFTRGVYYPDKVFRSSVLHSTQDLFLPFFSNVTWFHAIHVSGTNGTKRFDNPVLPFNDGVYFASTEKSNIIRGWIFGTTLDSKTQSLLIVNNATNVVIKVCEFQFCNYPFLGVYYHKNNKSWMESEFRVYSSANNCTFEYVSQPFLMDLEGKQGNFKNLSEFVFKNIDGYFKIYSKHTPINLVRDLPQGFSALEPLVDLPIGINITRFQTLLALHRSYLTPGDSSSGWTAGAAAYYVGYLQPRTFLLKYNENGTITDAVDCALDPLSETKCTLK

SEQ ID NO: 85 - protein, 560 aa, Artificial Sequence
  RBD-NTD-foldon(Gamma variant)
QCVNFTNRTQLPSAYTNSFTRGVYYPDKVFRSSVLHSTQDLFLPFFSNVTWFHAIHVSGTNGTKRFDNPVLPFNDGVYFASTEKSNIIRGWIFGTTLDSKTQSLLIVNNATNVVIKVCEFQFCNYPFLGVYYHKNNKSWMESEFRVYSSANNCTFEYVSQPFLMDLEGKQGNFKNLSEFVFKNIDGYFKIYSKHTPINLVRDLPQGFSALEPLVDLPIGINITRFQTLLALHRSYLTPGDSSSGWTAGAAAYYVGYLQPRTFLLKYNENGTITDAVDCALDPLSETKCTLKSFTVEKGIYQTSNFRVQPTESIVRFPNITNLCPFGEVFNATRFASVYAWNRKRISNCVADYSVLYNSASFSTFKCYGVSPTKLNDLCFTNVYADSFVIRGDEVRQIAPGQTGTIADYNYKLPDDFTGCVIAWNSNNLDSKVGGNYNYLYRLFRKSNLKPFERDISTEIYQAGSTPCNGVKGFNCYFPLQSYGFQPTYGVGYQPYRVVVLSFELLHAPATVCGPKKSTNLVKNKCVNFGSGSGYIPEAPRDGQAYVRKDGEWVLLSTFLG

SEQ ID NO: 86 - protein, 255 aa, Artificial Sequence
  RBD-foldon Gamma variant
RVQPTESIVRFPNITNLCPFGEVFNATRFASVYAWNRKRISNCVADYSVLYNSASFSTFKCYGVSPTKLNDLCFTNVYADSFVIRGDEVRQIAPGQTGTIADYNYKLPDDFTGCVIAWNSNNLDSKVGGNYNYLYRLFRKSNLKPFERDISTEIYQAGSTPCNGVKGFNCYFPLQSYGFQPTYGVGYQPYRVVVLSFELLHAPATVCGPKKSTNLVKNKCVNFGSGSGYIPEAPRDGQAYVRKDGEWVLLSTFLG

SEQ ID NO: 87 - protein, 323 aa, Artificial Sequence
  NTD-foldon Gamma variant
QCVNFTNRTQLPSAYTNSFTRGVYYPDKVFRSSVLHSTQDLFLPFFSNVTWFHAIHVSGTNGTKRFDNPVLPFNDGVYFASTEKSNIIRGWIFGTTLDSKTQSLLIVNNATNVVIKVCEFQFCNYPFLGVYYHKNNKSWMESEFRVYSSANNCTFEYVSQPFLMDLEGKQGNFKNLSEFVFKNIDGYFKIYSKHTPINLVRDLPQGFSALEPLVDLPIGINITRFQTLLALHRSYLTPGDSSSGWTAGAAAYYVGYLQPRTFLLKYNENGTITDAVDCALDPLSETKCTLKGSGSGYIPEAPRDGQAYVRKDGEWVLLSTFLG

SEQ ID NO: 88 - protein, 1273 aa, Artificial Sequence
  Gamma501Y.V3 Surface glycoprotein
MFVFLVLLPLVSSQCVNFTNRTQLPSAYTNSFTRGVYYPDKVFRSSVLHSTQDLFLPFFSNVTWFHAIHVSGTNGTKRFDNPVLPFNDGVYFASTEKSNIIRGWIFGTTLDSKTQSLLIVNNATNVVIKVCEFQFCNYPFLGVYYHKNNKSWMESEFRVYSSANNCTFEYVSQPFLMDLEGKQGNFKNLSEFVFKNIDGYFKIYSKHTPINLVRDLPQGFSALEPLVDLPIGINITRFQTLLALHRSYLTPGDSSSGWTAGAAAYYVGYLQPRTFLLKYNENGTITDAVDCALDPLSETKCTLKSFTVEKGIYQTSNFRVQPTESIVRFPNITNLCPFGEVFNATRFASVYAWNRKRISNCVADYSVLYNSASFSTFKCYGVSPTKLNDLCFTNVYADSFVIRGDEVRQIAPGQTGTIADYNYKLPDDFTGCVIAWNSNNLDSKVGGNYNYLYRLFRKSNLKPFERDISTEIYQAGSTPCNGVKGFNCYFPLQSYGFQPTYGVGYQPYRVVVLSFELLHAPATVCGPKKSTNLVKNKCVNFNFNGLTGTGVLTESNKKFLPFQQFGRDIADTTDAVRDPQTLEILDITPCSFGGVSVITPGTNTSNQVAVLYQGVNCTEVPVAIHADQLTPTWRVYSTGSNVFQTRAGCLIGAEYVNNSYECDIPIGAGICASYQTQTNSPRRARSVASQSIIAYTMSLGAENSVAYSNNSIAIPTNFTISVTTEILPVSMTKTSVDCTMYICGDSTECSNLLLQYGSFCTQLNRALTGIAVEQDKNTQEVFAQVKQIYKTPPIKDFGGFNFSQILPDPSKPSKRSFIEDLLFNKVTLADAGFIKQYGDCLGDIAARDLICAQKFNGLTVLPPLLTDEMIAQYTSALLAGTITSGWTFGAGAALQIPFAMQMAYRFNGIGVTQNVLYENQKLIANQFNSAIGKIQDSLSSTASALGKLQDVVNQNAQALNTLVKQLSSNFGAISSVLNDILSRLDKVEAEVQIDRLITGRLQSLQTYVTQQLIRAAEIRASANLAAIKMSECVLGQSKRVDFCGKGYHLMSFPQSAPHGVVFLHVTYVPAQEKNFTTAPAICHDGKAHFPREGVFVSNGTHWFVTQRNFYEPQIITTDNTFVSGNCDVVIGIVNNTVYDPLQPELDSFKEELDKYFKNHTSPDVDLGDISGINASFVNIQKEIDRLNEVAKNLNESLIDLQELGKYEQYIKWPWYIWLGFIAGLIAIVMVTIMLCCMTSCCSCLKGCCSCGSCCKFDEDDSEPVLKGVKLHYT

SEQ ID NO: 89 - protein, 5 aa, Artificial Sequence
  flexible linker
GSGSG

SEQ ID NO: 90 - protein, 14 aa, Artificial Sequence
  linker sequence
SFTVEKGIYQTSNF

SEQ ID NO: 91 - protein, 19 aa, Artificial Sequence
  signal peptide_3
MGWSCIILFLVATATGVHS

SEQ ID NO: 92 - protein, 566 aa, Artificial Sequence
  A type(H1N1)
MKAILVVMLYTFTTANADTLCIGYHANNSTDTVDTVLEKNVTVTHSVNLLEDKHNGKLCKLRGVAPLHLGKCNIAGWILGNPECESLSTARSWSYIVETSNSDNGTCYPGDFINYEELREQLSSVSSFERFEIFPKTSSWPNHDSDNGVTAACPHAGAKSFYKNLIWLVKKGKSYPKINQTYINDKGKEVLVLWGIHHPPTIADQQSLYQNADAYVFVGTSRYSKKFKPEIATRPKVRDQEGRMNYYWTLVEPGDKITFEATGNLVAPRYAFTMERDAGSGIIISDTPVHDCNTTCQTPEGAINTSLPFQNVHPITIGKCPKYVKSTKLRLATGLRNVPSIQSRGLFGAIAGFIEGGWTGMVDGWYGYHHQNEQGSGYAADLKSTQNAIDKITNKVNSVIEKMNTQFTAVGKEFNHLEKRIENLNKKVDDGFLDIWTYNAELLVLLENERTLDYHDSNVKNLYEKVRNQLKNNAKEIGNGCFEFYHKCDNTCMESVKNGTYDYPKYSEEAKLNREKIDGVKLDSTRIYQILAIYSTVASSLVLVVSLGAISFWMCSNGSLQCRICI

SEQ ID NO: 93 - protein, 566 aa, Artificial Sequence [sequence omitted]

SEQ ID NO: 94 - protein, 582 aa, Artificial Sequence
  B type(B/Washington/02/2019)
MKAIIVLLMVVTSNADRICTGITSSNSPHVVKTATQGEVNVTGVIPLTTTPTKSHFANLKGTETRGKLCPKCLNCTDLDVALGRPKCTGKIPSARVSILHEVRPVTSGCFPIMHDRTKIRQLPNLLRGYEHVRLSTHNVINAEDAPGRPYEIGTSGSCPNITNGNGFFATMAWAVPKNKTATNPLTIEVPYICTEGEDQITVWGFHSDNETQMAKLYGDSKPQKFTSSANGVTTHYVSQIGGFPNQTEDGGLPQSGRIVVDYMVQKSGKTGTITYQRGILLPQKVWCASGRSKVIKGSLPLIGEADCLHEKYGGLNKSKPYYTGEHAKAIGNCPIWVKTPLKLANGTKYRPPAKLLKERGFFGAIAGFLEGGWEGMIAGWHGYTSHGAHGVAVAADLKSTQEAINKITKNLNSLSELEVKNLQRLSGAMDELHNEILELDEKVDDLRADTISSQIELAVLLSNEGIINSEDEHLLALERKLKKMLGPSAVEIGNGCFETKHKCNQTCLDRIAAGTFDAGEFSLPTFDSLNITAASLNDDGLDNHTILLYYSTAASSLAVTLMIAIFVVYMVSRDNVSCSICL

SEQ ID NO: 95 - protein, 584 aa, Artificial Sequence
  B type(B/PHUKET/3073/2013)
MKAIIVLLMVVTSNADRICTGITSSNSPHVVKTATQGEVNVTGVIPLTTTPTKSYFANLKGTRTRGKLCPDCLNCTDLDVALGRPMCVGTTPSAKASILHEVRPVTSGCFPIMHDRTKIRQLPNLLRGYEKIRLSTQNVIDAEKAPGGPYRLGTSGSCPNATSKIGFFATMAWAVPKDNYKNATNPLTVEVPYICTEGEDQITVWGFHSDNKTQMKSLYGDSNPQKFTSSANGVTTHYVSQIGDFPDQTEDGGLPQSGRIVVDYMMQKPGKTGTIVYQRGVLLPQKVWCASGRSKVIKGSLPLIGEADCLHEEYGGLNKSKPYYTGKHAKAIGNCPIWVKTPLKLANGTKYRPPAKLLKERGFFGAIAGFLEGGWEGMIAGWHGYTSHGAHGVAVAADLKSTQEAINKITKNLNSLSELEVKNLQRLSGAMDELHNEILELDEKVDDLRADTISSQIELAVLLSNEGIINSEDEHLLALERKLKKMLGPSAVDIGNGCFETKHKCNQTCLDRIAAGTFNAGEFSLPTFDSLNITAASLNDDGLDNHTILLYYSTAASSLAVTLMLAIFIVYMVSRDNVSCSICL

SEQ ID NO: 96 - protein, 579 aa, Artificial Sequence
  RBD-NTD-foldon(WIV04)
MGWSCIILFLVATATGVHSQCVNLTTRTQLPPAYTNSFTRGVYYPDKVFRSSVLHSTQDLFLPFFSNVTWFHAIHVSGTNGTKRFDNPVLPFNDGVYFASTEKSNIIRGWIFGTTLDSKTQSLLIVNNATNVVIKVCEFQFCNDPFLGVYYHKNNKSWMESEFRVYSSANNCTFEYVSQPFLMDLEGKQGNFKNLREFVFKNIDGYFKIYSKHTPINLVRDLPQGFSALEPLVDLPIGINITRFQTLLALHRSYLTPGDSSSGWTAGAAAYYVGYLQPRTFLLKYNENGTITDAVDCALDPLSETKCTLKSFTVEKGIYQTSNFRVQPTESIVRFPNITNLCPFGEVFNATRFASVYAWNRKRISNCVADYSVLYNSASFSTFKCYGVSPTKLNDLCFTNVYADSFVIRGDEVRQIAPGQTGKIADYNYKLPDDFTGCVIAWNSNNLDSKVGGNYNYLYRLFRKSNLKPFERDISTEIYQAGSTPCNGVEGFNCYFPLQSYGFQPTNGVGYQPYRVVVLSFELLHAPATVCGPKKSTNLVKNKCVNFGSGSGYIPEAPRDGQAYVRKDGEWVLLSTFLG

SEQ ID NO: 97 - protein, 219 aa, Artificial Sequence
  RBD(WH)8Cys
RVQPTESIVRFPNITNLCPFGEVFNATRFASVYAWNRKRISNCVADYSVLYNSASFSTFKCYGVSPTKLNDLCFTNVYADSFVIRGDEVRQIAPGQTGKIADYNYKLPDDFTGCVIAWNSNNLDSKVGGNYNYLYRLFRKSNLKPFERDISTEIYQAGSTPCNGVEGFNCYFPLQSYGFQPTNGVGYQPYRVVVLSFELLHAPATVCGPKKSTNLVKNK

SEQ ID NO: 98 - protein, 248 aa, Artificial Sequence
  RBD(WH)10Cys(Add 2 to the N terminal)
DCALDPLSETKCTLKSFTVEKGIYQTSNFRVQPTESIVRFPNITNLCPFGEVFNATRFASVYAWNRKRISNCVADYSVLYNSASFSTFKCYGVSPTKLNDLCFTNVYADSFVIRGDEVRQIAPGQTGKIADYNYKLPDDFTGCVIAWNSNNLDSKVGGNYNYLYRLFRKSNLKPFERDISTEIYQAGSTPCNGVEGFNCYFPLQSYGFQPTNGVGYQPYRVVVLSFELLHAPATVCGPKKSTNLVKNK

SEQ ID NO: 99 - protein, 274 aa, Artificial Sequence
  RBD(WH)10Cys(Add 2 to the C terminal)
RVQPTESIVRFPNITNLCPFGEVFNATRFASVYAWNRKRISNCVADYSVLYNSASFSTFKCYGVSPTKLNDLCFTNVYADSFVIRGDEVRQIAPGQTGKIADYNYKLPDDFTGCVIAWNSNNLDSKVGGNYNYLYRLFRKSNLKPFERDISTEIYQAGSTPCNGVEGFNCYFPLQSYGFQPTNGVGYQPYRVVVLSFELLHAPATVCGPKKSTNLVKNKCVNFNFNGLTGTGVLTESNKKFLPFQQFGRDIADTTDAVRDPQTLEILDITPCSF

SEQ ID NO: 100 - protein, 303 aa, Artificial Sequence
  RBD(WH)12Cys(Add two to the N terminal and two to the C terminal)
DCALDPLSETKCTLKSFTVEKGIYQTSNFRVQPTESIVRFPNITNLCPFGEVFNATRFASVYAWNRKRISNCVADYSVLYNSASFSTFKCYGVSPTKLNDLCFTNVYADSFVIRGDEVRQIAPGQTGKIADYNYKLPDDFTGCVIAWNSNNLDSKVGGNYNYLYRLFRKSNLKPFERDISTEIYQAGSTPCNGVEGFNCYFPLQSYGFQPTNGVGYQPYRVVVLSFELLHAPATVCGPKKSTNLVKNKCVNFNFNGLTGTGVLTESNKKFLPFQQFGRDIADTTDAVRDPQTLEILDITPCSF

SEQ ID NO: 101 - protein, 219 aa, Artificial Sequence
  RBD(Africa)8Cys
RVQPTESIVRFPNITNLCPFGEVFNATRFASVYAWNRKRISNCVADYSVLYNSASFSTFKCYGVSPTKLNDLCFTNVYADSFVIRGDEVRQIAPGQTGNIADYNYKLPDDFTGCVIAWNSNNLDSKVGGNYNYLYRLFRKSNLKPFERDISTEIYQAGSTPCNGVKGFNCYFPLQSYGFQPTYGVGYQPYRVVVLSFELLHAPATVCGPKKSTNLVKNK

SEQ ID NO: 102 - protein, 248 aa, Artificial Sequence
  RBD(Africa)10Cys(Add 2 to the N terminal)
DCALDPLSETKCTLKSFTVEKGIYQTSNFRVQPTESIVRFPNITNLCPFGEVFNATRFASVYAWNRKRISNCVADYSVLYNSASFSTFKCYGVSPTKLNDLCFTNVYADSFVIRGDEVRQIAPGQTGNIADYNYKLPDDFTGCVIAWNSNNLDSKVGGNYNYLYRLFRKSNLKPFERDISTEIYQAGSTPCNGVKGFNCYFPLQSYGFQPTYGVGYQPYRVVVLSFELLHAPATVCGPKKSTNLVKNK

SEQ ID NO: 103 - protein, 274 aa, Artificial Sequence
  RBD(Africa)10Cys(Add 2 to the C terminal)
RVQPTESIVRFPNITNLCPFGEVFNATRFASVYAWNRKRISNCVADYSVLYNSASFSTFKCYGVSPTKLNDLCFTNVYADSFVIRGDEVRQIAPGQTGNIADYNYKLPDDFTGCVIAWNSNNLDSKVGGNYNYLYRLFRKSNLKPFERDISTEIYQAGSTPCNGVKGFNCYFPLQSYGFQPTYGVGYQPYRVVVLSFELLHAPATVCGPKKSTNLVKNKCVNFNFNGLTGTGVLTESNKKFLPFQQFGRDIADTTDAVRDPQTLEILDITPCSF

SEQ ID NO: 104 - protein, 303 aa, Artificial Sequence
  RBD(Africa)12Cys(Add 2 to the N terminal and add 2 to the C terminal)
DCALDPLSETKCTLKSFTVEKGIYQTSNFRVQPTESIVRFPNITNLCPFGEVFNATRFASVYAWNRKRISNCVADYSVLYNSASFSTFKCYGVSPTKLNDLCFTNVYADSFVIRGDEVRQIAPGQTGNIADYNYKLPDDFTGCVIAWNSNNLDSKVGGNYNYLYRLFRKSNLKPFERDISTEIYQAGSTPCNGVKGFNCYFPLQSYGFQPTYGVGYQPYRVVVLSFELLHAPATVCGPKKSTNLVKNKCVNFNFNGLTGTGVLTESNKKFLPFQQFGRDIADTTDAVRDPQTLEILDITPCSF

SEQ ID NO: 105 - protein, 219 aa, Artificial Sequence
  RBD(Delta)8Cys
RVQPTESIVRFPNITNLCPFGEVFNATRFASVYAWNRKRISNCVADYSVLYNSASFSTFKCYGVSPTKLNDLCFTNVYADSFVIRGDEVRQIAPGQTGKIADYNYKLPDDFTGCVIAWNSNNLDSKVGGNYNYRYRLFRKSNLKPFERDISTEIYQAGSKPCNGVEGFNCYFPLQSYGFQPTNGVGYQPYRVVVLSFELLHAPATVCGPKKSTNLVKNK

SEQ ID NO: 106 - protein, 248 aa, Artificial Sequence
  RBD(Delta)10Cys(Add 3 to the N terminal)
DCALDPLSETKCTLKSFTVEKGIYQTSNFRVQPTESIVRFPNITNLCPFGEVFNATRFASVYAWNRKRISNCVADYSVLYNSASFSTFKCYGVSPTKLNDLCFTNVYADSFVIRGDEVRQIAPGQTGKIADYNYKLPDDFTGCVIAWNSNNLDSKVGGNYNYRYRLFRKSNLKPFERDISTEIYQAGSKPCNGVEGFNCYFPLQSYGFQPTNGVGYQPYRVVVLSFELLHAPATVCGPKKSTNLVKNK

SEQ ID NO: 107 - protein, 274 aa, Artificial Sequence
  RBD(Delta)10Cys(Add 2 to the C terminal)
RVQPTESIVRFPNITNLCPFGEVFNATRFASVYAWNRKRISNCVADYSVLYNSASFSTFKCYGVSPTKLNDLCFTNVYADSFVIRGDEVRQIAPGQTGKIADYNYKLPDDFTGCVIAWNSNNLDSKVGGNYNYRYRLFRKSNLKPFERDISTEIYQAGSKPCNGVEGFNCYFPLQSYGFQPTNGVGYQPYRVVVLSFELLHAPATVCGPKKSTNLVKNKCVNFNFNGLTGTGVLTESNKKFLPFQQFGRDIADTTDAVRDPQTLEILDITPCSF

SEQ ID NO: 108 - protein, 303 aa, Artificial Sequence
  RBD(Delta)12Cys(Add 2 to the N terminal and add 2 to the C terminal)
DCALDPLSETKCTLKSFTVEKGIYQTSNFRVQPTESIVRFPNITNLCPFGEVFNATRFASVYAWNRKRISNCVADYSVLYNSASFSTFKCYGVSPTKLNDLCFTNVYADSFVIRGDEVRQIAPGQTGKIADYNYKLPDDFTGCVIAWNSNNLDSKVGGNYNYRYRLFRKSNLKPFERDISTEIYQAGSKPCNGVEGFNCYFPLQSYGFQPTNGVGYQPYRVVVLSFELLHAPATVCGPKKSTNLVKNKCVNFNFNGLTGTGVLTESNKKFLPFQQFGRDIADTTDAVRDPQTLEILDITPCSF

SEQ ID NO: 109 - protein, 305 aa, Artificial Sequence
  NTD(WH)
QCVNLTTRTQLPPAYTNSFTRGVYYPDKVFRSSVLHSTQDLFLPFFSNVTWFHAIHVSGTNGTKRFDNPVLPFNDGVYFASTEKSNIIRGWIFGTTLDSKTQSLLIVNNATNVVIKVCEFQFCNDPFLGVYYHKNNKSWMESEFRVYSSANNCTFEYVSQPFLMDLEGKQGNFKNLREFVFKNIDGYFKIYSKHTPINLVRDLPQGFSALEPLVDLPIGINITRFQTLLALHRSYLTPGDSSSGWTAGAAAYYVGYLQPRTFLLKYNENGTITDAVDCALDPLSETKCTLKSFTVEKGIYQTSNF

SEQ ID NO: 110 - protein, 302 aa, Artificial Sequence
  NTD(Africa)
QCVNFTTRTQLPPAYTNSFTRGVYYPDKVFRSSVLHSTQDLFLPFFSNVTWFHAIHVSGTNGTKRFANPVLPFNDGVYFASTEKSNIIRGWIFGTTLDSKTQSLLIVNNATNVVIKVCEFQFCNDPFLGVYYHKNNKSWMESEFRVYSSANNCTFEYVSQPFLMDLEGKQGNFKNLREFVFKNIDGYFKIYSKHTPINLVRGLPQGFSALEPLVDLPIGINITRFQTLHISYLTPGDSSSGWTAGAAAYYVGYLQPRTFLLKYNENGTITDAVDCALDPLSETKCTLKSFTVEKGIYQTSNF

SEQ ID NO: 111 - protein, 303 aa, Artificial Sequence
  NTD(Delta)
QCVNLRTRTQLPPAYTNSFTRGVYYPDKVFRSSVLHSTQDLFLPFFSNVTWFHAIHVSGTNGTKRFDNPVLPFNDGVYFASIEKSNIIRGWIFGTTLDSKTQSLLIVNNATNVVIKVCEFQFCNDPFLDVYYHKNNKSWMESGVYSSANNCTFEYVSQPFLMDLEGKQGNFKNLREFVFKNIDGYFKIYSKHTPINLVRDLPQGFSALEPLVDLPIGINITRFQTLLALHRSYLTPGDSSSGWTAGAAAYYVGYLQPRTFLLKYNENGTITDAVDCALDPLSETKCTLKSFTVEKGIYQTSNF